European Patent Application EP 4 567 111 A2, published June 11, 2025. Title: COMPOSITION FOR CLEAVING A TARGET DNA COMPRISING A GUIDE RNA SPECIFIC FOR THE TARGET DNA AND CAS PROTEIN-ENCODING NUCLEIC ACID OR CAS PROTEIN, AND USE THEREOF. Applicant: Toolgen Incorporated. Application EP. The sequence listing filed with the application follows.

SEQUENCE LISTING (297 sequences)

SEQ ID NO: 1 - DNA, 4107 bp, synthetic construct
  misc_feature 1..4107: note = Description of Artificial Sequence: Synthetic polynucleotide
  misc_feature 1..4107: note = Cas9-coding sequence
  source 1..4107: mol_type = other DNA
atggacaagaagtacagcatcggcctggacatcggtaccaacagcgtgggctgggccgtgatcaccgacgagtacaaggtgcccagcaagaagttcaaggtgctgggcaacaccgaccgccacagcatcaagaagaacctgatcggcgccctgctgttcgacagcggcgagaccgccgaggccacccgcctgaagcgcaccgcccgccgccgctacacccgccgcaagaaccgcatctgctacctgcaggagatcttcagcaacgagatggccaaggtggacgacagcttcttccaccgcctggaggagagcttcctggtggaggaggacaagaagcacgagcgccaccccatcttcggcaacatcgtggacgaggtggcctaccacgagaagtaccccaccatctaccacctgcgcaagaagctggtggacagcaccgacaaggccgacctgcgcctgatctacctggccctggcccacatgatcaagttccgcggccacttcctgatcgagggcgacctgaaccccgacaacagcgacgtggacaagctgttcatccagctggtgcagacctacaaccagctgttcgaggagaaccccatcaacgccagcggcgtggacgccaaggccatcctgagcgcccgcctgagcaagagccgccgcctggagaacctgatcgcccagctgcccggcgagaagaagaacggcctgttcggcaacctgatcgccctgagcctgggcctgacccccaacttcaagagcaacttcgacctggccgaggacgccaagctgcagctgagcaaggacacctacgacgacgacctggacaacctgctggcccagatcggcgaccagtacgccgacctgttcctggccgccaagaacctgagcgacgccatcctgctgagcgacatcctgcgcgtgaacaccgagatcaccaaggcccccctgagcgccagcatgatcaagcgctacgacgagcaccaccaggacctgaccctgctgaaggccctggtgcgccagcagctgcccgagaagtacaaggagatcttcttcgaccagagcaagaacggctacgccggctacatcgacggcggcgccagccaggaggagttctacaagttcatcaagcccatcctggagaagatggacggcaccgaggagctgctggtgaagctgaaccgcgaggacctgctgcgcaagcagcgcaccttcgacaacggcagcatcccccaccagatccacctgggcgagctgcacgccatcctgcgccgccaggaggacttctaccccttcctgaaggacaaccgcgagaagatcgagaagatcctgaccttccgcatcccctactacgtgggccccctggcccgcggcaacagccgcttcgcctggatgacccgcaagagcgaggagaccatcaccccctggaacttcgaggaggtggtggacaagggcgccagcgcccagagcttcatcgagcgcatgaccaacttcgacaagaacctgcccaacgagaaggtgctgcccaagcacagcctgctgtacgagtacttcaccgtgtacaacgagctgaccaaggtgaagtacgtgaccgagggcatgcgcaagcccgccttcctgagcggcgagcagaagaaggccatcgtggacctgctgttcaagaccaaccgcaaggtgaccgtgaagcagctgaaggaggactacttcaagaagatcgagtgcttcgacagcgtggagatcagcggcgtggaggaccgcttcaacgccagcctgggcacctaccacgacctgctgaagatcatcaaggacaaggacttcctggacaacgaggagaacgaggacatcctggaggacatcgtgctgaccctgaccctgttcgaggaccgcgagatgatcgaggagcgcctgaagacctacgcccacctgttcgacgacaaggtgatgaagcagctgaagcgccgccgctacaccggctggggccgcctgagccgcaagcttatcaacggcatccgcgacaagcagagcggcaagaccatcctggacttcctgaagagcgacggcttcgccaaccgcaacttcatgcagctgatccacgacgacagcctgaccttcaaggaggacatccagaaggcccaggtgagcggccagggcgacagcctgcacgagcacatcgccaacctggccggcagccccgccatcaagaagggcatcctgcagaccgtgaaggtggtggacgagctggtgaaggtgatgggccgccacaagcccgagaacatcgtgatcgagatggcccgcgagaaccagaccacccagaagggccagaagaacagccgcgagcgcatgaagcgcatcgaggagggcatcaaggagctgggcagccagatcctgaaggagcaccccgtggagaacacccagctgcagaacgagaagctgtacctgtactacctgcagaacggccgcgacatgtacgtggaccaggagctggacatcaaccgcctgagcgactacgacgtggaccacatcgtgccccagagcttcctgaaggacgacagcatcgacaacaaggtgctgacccgcagcgacaagaaccgcggcaagagcgacaacgtgcccagcgaggaggtggtgaagaagatgaagaactactggcgccagctgctgaacgccaagctgatcacccagcgcaagttcgacaacctgaccaaggccgagcgcggcggcctgagcgagctggacaaggccggcttcatcaagcgccagctggtggagacccgccagatcaccaagcacgtggcccagatcctggacagccgcatgaacaccaagtacgacgagaacgacaagctgatccgcgaggtgaaggtgatcaccctgaagagcaagctggtgagcgacttccgcaaggacttccagttctacaaggtgcgcgagatcaacaactaccaccacgcccacgacgcctacctgaacgccgtggtgggcaccgccctgatcaagaagtaccccaagctggagagcgagttcgtgtacggcgactacaaggtgtacgacgtgcgcaagatgatcgccaagagcgagcaggagatcggcaaggccaccgccaagtacttcttctacagcaacatcatgaacttcttcaagaccgagatcaccctggccaacggcgagatccgcaagcgccccctgatcgagaccaacggcgagaccggcgagatcgtgtgggacaagggccgcgacttcgccaccgtgcgcaaggtgctgagcatgccccaggtgaacatcgtgaagaagaccgaggtgcagaccggcggcttcagcaaggagagcatcctgcccaagcgcaacagcgacaagctgatcgcccgcaagaaggactgggaccccaagaagtacggcggcttcgacagccccaccgtggcctacagcgtgctggtggtggccaaggtggagaagggcaagagcaagaagctgaagagcgtgaaggagctgctgggcatcaccatcatggagcgcagcagcttcgagaagaaccccatcgacttcctggaggccaagggctacaaggaggtgaagaaggacctgatcatcaagctgcccaagtacagcctgttcgagctggagaacggccgcaagcgcatgctggccagcgccggcgagctgcagaagggcaacgagctggccctgcccagcaagtacgtgaacttcctgtacctggccagccactacgagaagctgaagggcagccccgaggacaacgagcagaagcagctgttcgtggagcagcacaagcactacctggacgagatcatcgagcagatcagcgagttcagcaagcgcgtgatcctggccgacgccaacctggacaaggtgctgagcgcctacaacaagcaccgcgacaagcccatccgcgagcaggccgagaacatcatccacctgttcaccctgaccaacctgggcgcccccgccgccttcaagtacttcgacaccaccatcgaccgcaagcgctacaccagcaccaaggaggtgctggacgccaccctgatccaccagagcatcaccggtctgtacgagacccgcatcgacctgagccagctgggcggcgactaa

SEQ ID NO: 2 - protein, 21 aa, synthetic construct
  REGION 1..21: note = Description of Artificial Sequence: Synthetic peptide
  REGION 1..21: note = Peptide tag
GGSGPPKKKRKVYPYDVPDYA

SEQ ID NO: 3 - DNA, 34 bp, synthetic construct
  misc_feature 1..34: note = Description of Artificial Sequence: Synthetic oligonucleotide
  misc_feature 1..34: note = F primer for CCR5
  source 1..34: mol_type = other DNA
aattcatgacatcaattattatacatcggaggag

SEQ ID NO: 4 - DNA, 34 bp, synthetic construct
  misc_feature 1..34: note = Description of Artificial Sequence: Synthetic oligonucleotide
  misc_feature 1..34: note = R primer for CCR5
  source 1..34: mol_type = other DNA
gatcctcctccgatgtataataattgatgtcatg

SEQ ID NO: 5 - DNA, 20 bp, synthetic construct
  misc_feature 1..20: note = Description of Artificial Sequence: Synthetic oligonucleotide
  misc_feature 1..20: note = F1 primer for CCR5
  source 1..20: mol_type = other DNA
ctccatggtgctatagagca

SEQ ID NO: 6 - DNA, 21 bp, synthetic construct
  misc_feature 1..21: note = Description of Artificial Sequence: Synthetic oligonucleotide
  misc_feature 1..21: note = F2 primer for CCR5
  source 1..21: mol_type = other DNA
gagccaagctctccatctagt

SEQ ID NO: 7 - DNA, 20 bp, synthetic construct
  misc_feature 1..20: note = Description of Artificial Sequence: Synthetic oligonucleotide
  misc_feature 1..20: note = R primer for CCR5
  source 1..20: mol_type = other DNA
gccctgtcaagagttgacac

SEQ ID NO: 8 - DNA, 20 bp, synthetic construct
  misc_feature 1..20: note = Description of Artificial Sequence: Synthetic oligonucleotide
  misc_feature 1..20: note = F1 primer for C4BPB
  source 1..20: mol_type = other DNA
tatttggctggttgaaaggg

SEQ ID NO: 9 - DNA, 24 bp, synthetic construct
  misc_feature 1..24: note = Description of Artificial Sequence: Synthetic oligonucleotide
  misc_feature 1..24: note = R1 primer for C4BPB
  source 1..24: mol_type = other DNA
aaagtcatgaaataaacacaccca

SEQ ID NO: 10 - DNA, 24 bp, synthetic construct
  misc_feature 1..24: note = Description of Artificial Sequence: Synthetic oligonucleotide
  misc_feature 1..24: note = F2 primer for C4BPB
  source 1..24: mol_type = other DNA
ctgcattgatatggtagtaccatg

SEQ ID NO: 11 - DNA, 21 bp, synthetic construct
  misc_feature 1..21: note = Description of Artificial Sequence: Synthetic oligonucleotide
  misc_feature 1..21: note = R2 primer for C4BPB
  source 1..21: mol_type = other DNA
gctgttcattgcaatggaatg

SEQ ID NO: 12 - DNA, 20 bp, synthetic construct
  misc_feature 1..20: note = Description of Artificial Sequence: Synthetic oligonucleotide
  misc_feature 1..20: note = F1 primer for ADCY5
  source 1..20: mol_type = other DNA
gctcccaccttagtgctctg

SEQ ID NO: 13 - DNA, 20 bp, synthetic construct
  misc_feature 1..20: note = Description of Artificial Sequence: Synthetic oligonucleotide
  misc_feature 1..20: note = R1 primer for ADCY5
  source 1..20: mol_type = other DNA
ggtggcaggaacctgtatgt

SEQ ID NO: 14 - DNA, 21 bp, synthetic construct
  misc_feature 1..21: note = Description of Artificial Sequence: Synthetic oligonucleotide
  misc_feature 1..21: note = F2 primer for ADCY5
  source 1..21: mol_type = other DNA
gtcattggccagagatgtgga

SEQ ID NO: 15 - DNA, 20 bp, synthetic construct
  misc_feature 1..20: note = Description of Artificial Sequence: Synthetic oligonucleotide
  misc_feature 1..20: note = R2 primer for ADCY5
  source 1..20: mol_type = other DNA
gtcccatgacaggcgtgtat

SEQ ID NO: 16 - DNA, 20 bp, synthetic construct
  misc_feature 1..20: note = Description of Artificial Sequence: Synthetic oligonucleotide
  misc_feature 1..20: note = F primer for KCNJ6
  source 1..20: mol_type = other DNA
gcctggccaagtttcagtta

SEQ ID NO: 17 - DNA, 20 bp, synthetic construct
  misc_feature 1..20: note = Description of Artificial Sequence: Synthetic oligonucleotide
  misc_feature 1..20: note = R1 primer for KCNJ6
  source 1..20: mol_type = other DNA
tggagccattggtttgcatc

SEQ ID NO: 18 - DNA, 22 bp, synthetic construct
  misc_feature 1..22: note = Description of Artificial Sequence: Synthetic oligonucleotide
  misc_feature 1..22: note = R2 primer for KCNJ6
  source 1..22: mol_type = other DNA
ccagaactaagccgtttctgac

SEQ ID NO: 19 - DNA, 20 bp, synthetic construct
  misc_feature 1..20: note = Description of Artificial Sequence: Synthetic oligonucleotide
  misc_feature 1..20: note = F1 primer for CNTNAP2
  source 1..20: mol_type = other DNA
atcaccgacaaccagtttcc

SEQ ID NO: 20 - DNA, 20 bp, synthetic construct
  misc_feature 1..20: note = Description of Artificial Sequence: Synthetic oligonucleotide
  misc_feature 1..20: note = F2 primer for CNTNAP2
  source 1..20: mol_type = other DNA
tgcagtgcagactctttcca

SEQ ID NO: 21 - DNA, 20 bp, synthetic construct
  misc_feature 1..20: note = Description of Artificial Sequence: Synthetic oligonucleotide
  misc_feature 1..20: note = R primer for CNTNAP2
  source 1..20: mol_type = other DNA
aaggacacagggcaactgaa

SEQ ID NO: 22 - DNA, 20 bp, synthetic construct
  misc_feature 1..20: note = Description of Artificial Sequence: Synthetic oligonucleotide
  misc_feature 1..20: note = F1 primer for N/A Chr. 5
  source 1..20: mol_type = other DNA
tgtggaacgagtggtgacag

SEQ ID NO: 23 - DNA, 22 bp, synthetic construct
  misc_feature 1..22: note = Description of Artificial Sequence: Synthetic oligonucleotide
  misc_feature 1..22: note = R1 primer for N/A Chr. 5
  source 1..22: mol_type = other DNA
gctggattaggaggcaggattc

SEQ ID NO: 24 - DNA, 22 bp, synthetic construct
  misc_feature 1..22: note = Description of Artificial Sequence: Synthetic oligonucleotide
  misc_feature 1..22: note = F2 primer for N/A Chr. 5
  source 1..22: mol_type = other DNA
gtgctgagaacgcttcatagag

SEQ ID NO: 25 - DNA, 23 bp, synthetic construct
  misc_feature 1..23: note = Description of Artificial Sequence: Synthetic oligonucleotide
  misc_feature 1..23: note = R2 primer for N/A Chr. 5
  source 1..23: mol_type = other DNA
ggaccaaaccacattcttctcac

SEQ ID NO: 26 - DNA, 20 bp, synthetic construct
  misc_feature 1..20: note = Description of Artificial Sequence: Synthetic oligonucleotide
  misc_feature 1..20: note = F primer for deletion
  source 1..20: mol_type = other DNA
ccacatctcgttctcggttt

SEQ ID NO: 27 - DNA, 20 bp, synthetic construct
  misc_feature 1..20: note = Description of Artificial Sequence: Synthetic oligonucleotide
  misc_feature 1..20: note = R primer for deletion
  source 1..20: mol_type = other DNA
tcacaagcccacagatattt

SEQ ID NO: 28 - RNA, 105 nt, synthetic construct
  misc_feature 1..105: note = Description of Artificial Sequence: Synthetic polynucleotide
  misc_feature 1..105: note = sgRNA for CCR5
  source 1..105: mol_type = other RNA
ggtgacatcaattattatacatgttttagagctagaaatagcaagttaaaataaggctagtccgttatcaacttgaaaaagtggcaccgagtcggtgcttttttt

SEQ ID NO: 29 - RNA, 44 nt, synthetic construct
  misc_feature 1..44: note = Description of Artificial Sequence: Synthetic oligonucleotide
  misc_feature 1..44: note = crRNA for CCR5
  source 1..44: mol_type = other RNA
ggtgacatcaattattatacatgttttagagctatgctgttttg

SEQ ID NO: 30 - RNA, 86 nt, synthetic construct
  misc_feature 1..86: note = Description of Artificial Sequence: Synthetic oligonucleotide
  misc_feature 1..86: note = tracrRNA for CCR5
  source 1..86: mol_type = other RNA
ggaaccattcaaaacagcatagcaagttaaaataaggctagtccgttatcaacttgaaaaagtggcaccgagtcggtgcttttttt

SEQ ID NO: 31 - DNA, 86 bp, synthetic construct
  misc_feature 1..86: note = Description of Artificial Sequence: Synthetic oligonucleotide
  misc_feature 1..86: note = Foxn1 #1 sgRNA
  source 1..86: mol_type = other DNA
gaaattaatacgactcactataggcagtctgacgtcacacttccgttttagagctagaaatagcaagttaaaataaggctagtccg

SEQ ID NO: 32 - DNA, 86 bp, synthetic construct
  misc_feature 1..86: note = Description of Artificial Sequence: Synthetic oligonucleotide
  misc_feature 1..86: note = Foxn1 #2 sgRNA
  source 1..86: mol_type = other DNA
gaaattaatacgactcactataggacttccaggctccacccgacgttttagagctagaaatagcaagttaaaataaggctagtccg

SEQ ID NO: 33 - DNA, 86 bp, synthetic construct
  misc_feature 1..86: note = Description of Artificial Sequence: Synthetic oligonucleotide
  misc_feature 1..86: note = Foxn1 #3 sgRNA
  source 1..86: mol_type = other DNA
gaaattaatacgactcactataggccaggctccacccgactggagttttagagctagaaatagcaagttaaaataaggctagtccg

SEQ ID NO: 34 - DNA, 86 bp, synthetic construct
  misc_feature 1..86: note = Description of Artificial Sequence: Synthetic oligonucleotide
  misc_feature 1..86: note = Foxn1 #4 sgRNA
  source 1..86: mol_type = other DNA
gaaattaatacgactcactataggactggagggcgaaccccaaggttttagagctagaaatagcaagttaaaataaggctagtccg

SEQ ID NO: 35 - DNA, 86 bp, synthetic construct
  misc_feature 1..86: note = Description of Artificial Sequence: Synthetic oligonucleotide
  misc_feature 1..86: note = Foxn1 #5 sgRNA
  source 1..86: mol_type = other DNA
gaaattaatacgactcactataggaccccaaggggacctcatgcgttttagagctagaaatagcaagttaaaataaggctagtccg

SEQ ID NO: 36 - DNA, 86 bp, synthetic construct
  misc_feature 1..86: note = Description of Artificial Sequence: Synthetic oligonucleotide
  misc_feature 1..86: note = Prkdc #1 sgRNA
  source 1..86: mol_type = other DNA
gaaattaatacgactcactataggttagttttttccagagacttgttttagagctagaaatagcaagttaaaataaggctagtccg

SEQ ID NO: 37 - DNA, 86 bp, synthetic construct
  misc_feature 1..86: note = Description of Artificial Sequence: Synthetic oligonucleotide
  misc_feature 1..86: note = Prkdc #2 sgRNA
  source 1..86: mol_type = other DNA
gaaattaatacgactcactataggttggtttgcttgtgtttatcgttttagagctagaaatagcaagttaaaataaggctagtccg

SEQ ID NO: 38 - DNA, 86 bp, synthetic construct
  misc_feature 1..86: note = Description of Artificial Sequence: Synthetic oligonucleotide
  misc_feature 1..86: note = Prkdc #3 sgRNA
  source 1..86: mol_type = other DNA
gaaattaatacgactcactataggcacaagcaaaccaaagtctcgttttagagctagaaatagcaagttaaaataaggctagtccg

SEQ ID NO: 39 - DNA, 86 bp, synthetic construct
  misc_feature 1..86: note = Description of Artificial Sequence: Synthetic oligonucleotide
  misc_feature 1..86: note = Prkdc #4 sgRNA
  source 1..86: mol_type = other DNA
gaaattaatacgactcactataggcctcaatgctaagcgacttcgttttagagctagaaatagcaagttaaaataaggctagtccg

SEQ ID NO: 40 - DNA, 29 bp, synthetic construct
  misc_feature 1..29: note = Description of Artificial Sequence: Synthetic oligonucleotide
  misc_feature 1..29: note = F1 primer for Foxn1
  source 1..29: mol_type = other DNA
gtctgtctatcatctcttcccttctctcc

SEQ ID NO: 41 - DNA, 25 bp, synthetic construct
  misc_feature 1..25: note = Description of Artificial Sequence: Synthetic oligonucleotide
  misc_feature 1..25: note = F2 primer for Foxn1
  source 1..25: mol_type = other DNA
tccctaatccgatggctagctccag

SEQ ID NO: 42 - DNA, 23 bp, synthetic construct
  misc_feature 1..23: note = Description of Artificial Sequence: Synthetic oligonucleotide
  misc_feature 1..23: note = R1 primer for Foxn1
  source 1..23: mol_type = other DNA
acgagcagctgaagttagcatgc

SEQ ID NO: 43 - DNA, 32 bp, synthetic construct
  misc_feature 1..32: note = Description of Artificial Sequence: Synthetic oligonucleotide
  misc_feature 1..32: note = R2 primer for Foxn1
  source 1..32: mol_type = other DNA
ctactcaatgctcttagagctaccaggcttgc

SEQ ID NO: 44 - DNA, 20 bp, synthetic construct
  misc_feature 1..20: note = Description of Artificial Sequence: Synthetic oligonucleotide
  misc_feature 1..20: note = F primer for Prkdc
  source 1..20: mol_type = other DNA
gactgttgtggggagggccg

SEQ ID NO: 45 - DNA, 24 bp, synthetic construct
  misc_feature 1..24: note = Description of Artificial Sequence: Synthetic oligonucleotide
  misc_feature 1..24: note = F2 primer for Prkdc
  source 1..24: mol_type = other DNA
gggagggccgaaagtcttattttg

SEQ ID NO: 46 - DNA, 28 bp, synthetic construct
  misc_feature 1..28: note = Description of Artificial Sequence: Synthetic oligonucleotide
  misc_feature 1..28: note = R1 primer for Prkdc
  source 1..28: mol_type = other DNA
cctgaagactgaagttggcagaagtgag

SEQ ID NO: 47 - DNA, 27 bp, synthetic construct
  misc_feature 1..27: note = Description of Artificial Sequence: Synthetic oligonucleotide
  misc_feature 1..27: note = R2 primer for Prkdc
  source 1..27: mol_type = other DNA
ctttagggcttcttctctacaatcacg

SEQ ID NO: 48 - DNA, 38 bp, synthetic construct
  misc_feature 1..38: note = Description of Artificial Sequence: Synthetic oligonucleotide
  misc_feature 1..38: note = F primer for Foxn1
  source 1..38: mol_type = other DNA
ctcggtgtgtagccctgacctcggtgtgtagccctgac

SEQ ID NO: 49 - DNA, 21 bp, synthetic construct
  misc_feature 1..21: note = Description of Artificial Sequence: Synthetic oligonucleotide
  misc_feature 1..21: note = R primer for Foxn1
  source 1..21: mol_type = other DNA
agactggcctggaactcacag

SEQ ID NO: 50 - DNA, 23 bp, synthetic construct
  misc_feature 1..23: note = Description of Artificial Sequence: Synthetic oligonucleotide
  misc_feature 1..23: note = F primer for Foxn1
  source 1..23: mol_type = other DNA
cactaaagcctgtcaggaagccg

SEQ ID NO: 51 - DNA, 21 bp, synthetic construct
  misc_feature 1..21: note = Description of Artificial Sequence: Synthetic oligonucleotide
  misc_feature 1..21: note = R primer for Foxn1
  source 1..21: mol_type = other DNA
ctgtggagagcacacagcagc

SEQ ID NO: 52 - DNA, 19 bp, synthetic construct
  misc_feature 1..19: note = Description of Artificial Sequence: Synthetic oligonucleotide
  misc_feature 1..19: note = F primer for Foxn1
  source 1..19: mol_type = other DNA
gctgcgacctgagaccatg

SEQ ID NO: 53 - DNA, 26 bp, synthetic construct
  misc_feature 1..26: note = Description of Artificial Sequence: Synthetic oligonucleotide
  misc_feature 1..26: note = R primer for Foxn1
  source 1..26: mol_type = other DNA
cttcaatggcttcctgcttaggctac

SEQ ID NO: 54 - DNA, 23 bp, synthetic construct
  misc_feature 1..23: note = Description of Artificial Sequence: Synthetic oligonucleotide
  misc_feature 1..23: note = F primer for Foxn1
  source 1..23: mol_type = other DNA
ggttcagatgaggccatcctttc

SEQ ID NO: 55 - DNA, 24 bp, synthetic construct
  misc_feature 1..24: note = Description of Artificial Sequence: Synthetic oligonucleotide
  misc_feature 1..24: note = R primer for Foxn1
  source 1..24: mol_type = other DNA
cctgatctgcaggcttaacccttg

SEQ ID NO: 56 - DNA, 22 bp, synthetic construct
  misc_feature 1..22: note = Description of Artificial Sequence: Synthetic oligonucleotide
  misc_feature 1..22: note = F primer for Prkdc
  source 1..22: mol_type = other DNA
ctcacctgcacatcacatgtgg

SEQ ID NO: 57 - DNA, 20 bp, synthetic construct
  misc_feature 1..20: note = Description of Artificial Sequence: Synthetic oligonucleotide
  misc_feature 1..20: note = R primer for Prkdc
  source 1..20: mol_type = other DNA
ggcatccaccctatggggtc

SEQ ID NO: 58 - DNA, 25 bp, synthetic construct
  misc_feature 1..25: note = Description of Artificial Sequence: Synthetic oligonucleotide
  misc_feature 1..25: note = F primer for Prkdc
  source 1..25: mol_type = other DNA
gccttgacctagagcttaaagagcc

SEQ ID NO: 59 - DNA, 25 bp, synthetic construct
  misc_feature 1..25: note = Description of Artificial Sequence: Synthetic oligonucleotide
  misc_feature 1..25: note = R primer for Prkdc
  source 1..25: mol_type = other DNA
ggtcttgttagcaggaaggacactg

SEQ ID NO: 60 - DNA, 27 bp, synthetic construct
  misc_feature 1..27: note = Description of Artificial Sequence: Synthetic oligonucleotide
  misc_feature 1..27: note = F primer for Prkdc
  source 1..27: mol_type = other DNA
aaaactctgcttgatgggatatgtggg

SEQ ID NO: 61 - DNA, 26 bp, synthetic construct
  misc_feature 1..26: note = Description of Artificial Sequence: Synthetic oligonucleotide
  misc_feature 1..26: note = R primer for Prkdc
  source 1..26: mol_type = other DNA
ctctcactggttatctgtgctccttc

SEQ ID NO: 62 - DNA, 23 bp, synthetic construct
  misc_feature 1..23: note = Description of Artificial Sequence: Synthetic oligonucleotide
  misc_feature 1..23: note = F primer for Prkdc
  source 1..23: mol_type = other DNA
ggatcaataggtggtgggggatg

SEQ ID NO: 63 - DNA, 27 bp, synthetic construct
  misc_feature 1..27: note = Description of Artificial Sequence: Synthetic oligonucleotide
  misc_feature 1..27: note = R primer for Prkdc
  source 1..27: mol_type = other DNA
gtgaatgacacaatgtgacagcttcag

SEQ ID NO: 64 - DNA, 28 bp, synthetic construct
  misc_feature 1..28: note = Description of Artificial Sequence: Synthetic oligonucleotide
  misc_feature 1..28: note = F primer for Prkdc
  source 1..28: mol_type = other DNA
cacaagacagacctctcaacattcagtc

SEQ ID NO: 65 - DNA, 32 bp, synthetic construct
  misc_feature 1..32: note = Description of Artificial Sequence: Synthetic oligonucleotide
  misc_feature 1..32: note = R primer for Prkdc
  source 1..32: mol_type = other DNA
gtgcatgcatataatccattctgattgctctc

SEQ ID NO: 66 - DNA, 17 bp, synthetic construct
  misc_feature 1..17: note = Description of Artificial Sequence: Synthetic oligonucleotide
  misc_feature 1..17: note = F1 primer for Prkdc
  source 1..17: mol_type = other DNA
gggaggcagaggcaggt

SEQ ID NO: 67 - DNA, 23 bp, synthetic construct
  misc_feature 1..23: note = Description of Artificial Sequence: Synthetic oligonucleotide
  misc_feature 1..23: note = F2 primer for Prkdc
  source 1..23: mol_type = other DNA
ggatctctgtgagtttgaggcca

SEQ ID NO: 68 - DNA, 24 bp, synthetic construct
  misc_feature 1..24: note = Description of Artificial Sequence: Synthetic oligonucleotide
  misc_feature 1..24: note = R1 primer for Prkdc
  source 1..24: mol_type = other DNA
gctccagaactcactcttaggctc

SEQ ID NO: 69 - DNA, 20 bp, synthetic construct
  misc_feature 1..20: note = Description of Artificial Sequence: Synthetic oligonucleotide
  misc_feature 1..20: note = Primer for Foxn1
  source 1..20: mol_type = other DNA
ctactccctccgcagtctga

SEQ ID NO: 70 - DNA, 20 bp, synthetic construct
  misc_feature 1..20: note = Description of Artificial Sequence: Synthetic oligonucleotide
  misc_feature 1..20: note = Primer for Foxn1
  source 1..20: mol_type = other DNA
ccaggcctaggttccaggta

SEQ ID NO: 71 - DNA, 20 bp, synthetic construct
  misc_feature 1..20: note = Description of Artificial Sequence: Synthetic oligonucleotide
  misc_feature 1..20: note = Primer for Prkdc
  source 1..20: mol_type = other DNA
ccccagcattgcagatttcc

SEQ ID NO: 72 - DNA, 23 bp, synthetic construct
  misc_feature 1..23: note = Description of Artificial Sequence: Synthetic oligonucleotide
  misc_feature 1..23: note = Primer for Prkdc
  source 1..23: mol_type = other DNA
agggcttcttctctacaatcacg

SEQ ID NO: 73 - DNA, 86 bp, synthetic construct
  misc_feature 1..86: note = Description of Artificial Sequence: Synthetic oligonucleotide
  misc_feature 1..86: note = BRI1 target 1
  source 1..86: mol_type = other DNA
gaaattaatacgactcactataggtttgaaagatggaagcgcgggttttagagctagaaatagcaagttaaaataaggctagtccg

SEQ ID NO: 74 - DNA, 86 bp, synthetic construct
  misc_feature 1..86: note = Description of Artificial Sequence: Synthetic oligonucleotide
  misc_feature 1..86: note = BRI1 target 2
  source 1..86: mol_type = other DNA
gaaattaatacgactcactataggtgaaactaaactggtccacagttttagagctagaaatagcaagttaaaataaggctagtccg

SEQ ID NO: 75 - DNA, 64 bp, synthetic construct
  misc_feature 1..64: note = Description of Artificial Sequence: Synthetic oligonucleotide
  misc_feature 1..64: note = Universal
  source 1..64: mol_type = other DNA
aaaaaagcaccgactcggtgccactttttcaagttgataacggactagccttattttaacttgc

SEQ ID NO: 76 - DNA, 65 bp, synthetic construct
  misc_feature 1..65: note = Description of Artificial Sequence: Synthetic oligonucleotide
  misc_feature 1..65: note = Templates for crRNA
  modified_base 25..44: mod_base = OTHER; note = a, c, t, g, or unknown
  source 1..65: mol_type = other DNA
gaaattaatacgactcactataggnnnnnnnnnnnnnnnnnnnngttttagagctatgctgtttt

SEQ ID NO: 77 - DNA, 67 bp, synthetic construct
  misc_feature 1..67: note = Description of Artificial Sequence: Synthetic oligonucleotide
  misc_feature 1..67: note = tracrRNA
  source 1..67: mol_type = other DNA
gaaattaatacgactcactataggaaccattcaaaacagcatagcaagttaaaataaggctagtccg

SEQ ID NO: 78 - DNA, 69 bp, synthetic construct
  misc_feature 1..69: note = Description of Artificial Sequence: Synthetic oligonucleotide
  misc_feature 1..69: note = tracrRNA
  source 1..69: mol_type = other DNA
aaaaaaagcaccgactcggtgccactttttcaagttgataacggactagccttattttaacttgctatg

SEQ ID NO: 79 - DNA, 20 bp, synthetic construct
  misc_feature 1..20: note = Description of Artificial Sequence: Synthetic oligonucleotide
  misc_feature 1..20: note = Primer
  source 1..20: mol_type = other DNA
ctccatggtgctatagagca

SEQ ID NO: 80 - DNA, 21 bp, synthetic construct
  misc_feature 1..21: note = Description of Artificial Sequence: Synthetic oligonucleotide
  misc_feature 1..21: note = Primer
  source 1..21: mol_type = other DNA
gagccaagctctccatctagt

SEQ ID NO: 81 - DNA, 20 bp, synthetic construct
  misc_feature 1..20: note = Description of Artificial Sequence: Synthetic oligonucleotide
  misc_feature 1..20: note = Primer
  source 1..20: mol_type = other DNA
gccctgtcaagagttgacac

SEQ ID NO: 82 - DNA, 22 bp, synthetic construct
  misc_feature 1..22: note = Description of Artificial Sequence: Synthetic oligonucleotide
  misc_feature 1..22: note = Primer
  source 1..22: mol_type = other DNA
gcacagggtggaacaagatgga

SEQ ID NO: 83 - DNA, 24 bp, synthetic construct
  misc_feature 1..24: note = Description of Artificial Sequence: Synthetic oligonucleotide
  misc_feature 1..24: note = Primer
  source 1..24: mol_type = other DNA
gccaggtacctatcgattgtcagg

SEQ ID NO: 84 - DNA, 21 bp, synthetic construct
  misc_feature 1..21: note = Description of Artificial Sequence: Synthetic oligonucleotide
  misc_feature 1..21: note = Primer
  source 1..21: mol_type = other DNA
gagccaagctctccatctagt

SEQ ID NO: 85 - DNA, 20 bp, synthetic construct
  misc_feature 1..20: note = Description of Artificial Sequence: Synthetic oligonucleotide
  misc_feature 1..20: note = Primer
  source 1..20: mol_type = other DNA
actctgactgggtcaccagc

SEQ ID NO: 86 - DNA, 20 bp, synthetic construct
  misc_feature 1..20: note = Description of Artificial Sequence: Synthetic oligonucleotide
  misc_feature 1..20: note = Primer
  source 1..20: mol_type = other DNA
tatttggctggttgaaaggg

SEQ ID NO: 87 - DNA, 24 bp, synthetic construct
  misc_feature 1..24: note = Description of Artificial Sequence: Synthetic oligonucleotide
  misc_feature 1..24: note = Primer
  source 1..24: mol_type = other DNA
aaagtcatgaaataaacacaccca

SEQ ID NO: 88 - DNA, 24 bp, synthetic construct
  misc_feature 1..24: note = Description of Artificial Sequence: Synthetic oligonucleotide
  misc_feature 1..24: note = Primer
  source 1..24: mol_type = other DNA
ctgcattgatatggtagtaccatg

SEQ ID NO: 89 - DNA, 21 bp, synthetic construct
  misc_feature 1..21: note = Description of Artificial Sequence: Synthetic oligonucleotide
  misc_feature 1..21: note = Primer
  source 1..21: mol_type = other DNA
gctgttcattgcaatggaatg

SEQ ID NO: 90 - DNA, 22 bp, synthetic construct
  misc_feature 1..22: note = Description of Artificial Sequence: Synthetic oligonucleotide
  misc_feature 1..22: note = Primer
  source 1..22: mol_type = other DNA
atggagttggacatggccatgg

SEQ ID NO: 91 - DNA, 28 bp, synthetic construct
  misc_feature 1..28: note = Description of Artificial Sequence: Synthetic oligonucleotide
  misc_feature 1..28: note = Primer
  source 1..28: mol_type = other DNA
actcactatccacagttcagcatttacc

SEQ ID NO: 92 - DNA, 23 bp, synthetic construct
  misc_feature 1..23: note = Description of Artificial Sequence: Synthetic oligonucleotide
  misc_feature 1..23: note = Primer
  source 1..23: mol_type = other DNA
tggagatagctgtcagcaacttt

SEQ ID NO: 93 - DNA, 29 bp, synthetic construct
  misc_feature 1..29: note = Description of Artificial Sequence: Synthetic oligonucleotide
  misc_feature 1..29: note = Primer
  source 1..29: mol_type = other DNA
caacaaagcaaaggtaaagttggtaatag

SEQ ID NO: 94 - DNA, 25 bp, synthetic construct
  misc_feature 1..25: note = Description of Artificial Sequence: Synthetic oligonucleotide
  misc_feature 1..25: note = Primer
  source 1..25: mol_type = other DNA
ggtttcaggagatgtgttacaaggc

SEQ ID NO: 95 - DNA, 27 bp, synthetic construct
  misc_feature 1..27: note = Description of Artificial Sequence: Synthetic oligonucleotide
  misc_feature 1..27: note = Primer
  source 1..27: mol_type = other DNA
gattgtgcaattcctatgcaatcggtc

SEQ ID NO: 96 - DNA, 25 bp, synthetic construct
  misc_feature 1..25: note = Description of Artificial Sequence: Synthetic oligonucleotide
  misc_feature 1..25: note = Primer
  source 1..25: mol_type = other DNA
cactgggtacttaatctgtagcctc

SEQ ID NO: 97 - DNA, 23 bp, synthetic construct
  misc_feature 1..23: note = Description of Artificial Sequence: Synthetic oligonucleotide
  misc_feature 1..23: note = Primer
  source 1..23: mol_type = other DNA
ggttccaagtcattcccagtagc

SEQ ID NO: 98 - DNA, 30 bp, synthetic construct
  misc_feature 1..30: note = Description of Artificial Sequence: Synthetic oligonucleotide
  misc_feature 1..30: note = Primer
  source 1..30: mol_type = other DNA
catcactgcagttgtaggttataactatcc

SEQ ID NO: 99 - DNA, 26 bp, synthetic construct
  misc_feature 1..26: note = Description of Artificial Sequence: Synthetic oligonucleotide
  misc_feature 1..26: note = Primer
  source 1..26: mol_type = other DNA
ttgaaaaccacagatctggttgaacc

SEQ ID NO: 100 - DNA, 22 bp, synthetic construct
  misc_feature 1..22: note = Description of Artificial Sequence: Synthetic oligonucleotide
  misc_feature 1..22: note = Primer
  source 1..22: mol_type = other DNA
ggagtgccaagagaatatctgg

SEQ ID NO: 101 - DNA, 32 bp, synthetic construct
  misc_feature 1..32: note = Description of Artificial Sequence: Synthetic oligonucleotide
  misc_feature 1..32: note = Primer
  source 1..32: mol_type = other DNA
ctgaaactggtttcaaaatattcgttttaagg

SEQ ID NO: 102 - DNA, 22 bp, synthetic construct
  misc_feature 1..22: note = Description of Artificial Sequence: Synthetic oligonucleotide
  misc_feature 1..22: note = Primer
  source 1..22: mol_type = other DNA
gctctgtatgccctgtagtagg

SEQ ID NO: 103 - DNA, 22 bp, synthetic construct
  misc_feature 1..22: note = Description of Artificial Sequence: Synthetic oligonucleotide
  misc_feature 1..22: note = Primer
  source 1..22: mol_type = other DNA
tttgcatctgaccttacctttg

SEQ ID NO: 104 - DNA, 23 bp, synthetic construct
  misc_feature 1..23: note = Description of Artificial Sequence: Synthetic oligonucleotide
  misc_feature 1..23: note = Target sequence of RGEN
  source 1..23: mol_type = other DNA
aatgaccactacatcctcaaggg

SEQ ID NO: 105 - DNA, 23 bp, synthetic construct
  misc_feature 1..23: note = Description of Artificial Sequence: Synthetic oligonucleotide
  misc_feature 1..23: note = Target sequence of RGEN
  source 1..23: mol_type = other DNA
agatgatgtctcatcatcagagg

SEQ ID NO: 106 - DNA, 4170 bp, synthetic construct
  misc_feature 1..4170: note = Description of Artificial Sequence: Synthetic polynucleotide
  misc_feature 1..4170: note = Cas9-coding sequence in p3s-Cas9HC (humanized, C-term tagging, human cell experiments)
  source 1..4170: mol_type = other DNA
atggacaagaagtacagcatcggcctggacatcggtaccaacagcgtgggctgggccgtgatcaccgacgagtacaaggtgcccagcaagaagttcaaggtgctgggcaacaccgaccgccacagcatcaagaagaacctgatcggcgccctgctgttcgacagcggcgagaccgccgaggccacccgcctgaagcgcaccgcccgccgccgctacacccgccgcaagaaccgcatctgctacctgcaggagatcttcagcaacgagatggccaaggtggacgacagcttcttccaccgcctggaggagagcttcctggtggaggaggacaagaagcacgagcgccaccccatcttcggcaacatcgtggacgaggtggcctaccacgagaagtaccccaccatctaccacctgcgcaagaagctggtggacagcaccgacaaggccgacctgcgcctgatctacctggccctggcccacatgatcaagttccgcggccacttcctgatcgagggcgacctgaaccccgacaacagcgacgtggacaagctgttcatccagctggtgcagacctacaaccagctgttcgaggagaaccccatcaacgccagcggcgtggacgccaaggccatcctgagcgcccgcctgagcaagagccgccgcctggagaacctgatcgcccagctgcccggcgagaagaagaacggcctgttcggcaacctgatcgccctgagcctgggcctgacccccaacttcaagagcaacttcgacctggccgaggacgccaagctgcagctgagcaaggacacctacgacgacgacctggacaacctgctggcccagatcggcgaccagtacgccgacctgttcctggccgccaagaacctgagcgacgccatcctgctgagcgacatcctgcgcgtgaacaccgagatcaccaaggcccccctgagcgccagcatgatcaagcgctacgacgagcaccaccaggacctgaccctgctgaaggccctggtgcgccagcagctgcccgagaagtacaaggagatcttcttcgaccagagcaagaacggctacgccggctacatcgacggcggcgccagccaggaggagttctacaagttcatcaagcccatcctggagaagatggacggcaccgaggagctgctggtgaagctgaaccgcgaggacctgctgcgcaagcagcgcaccttcgacaacggcagcatcccccaccagatccacctgggcgagctgcacgccatcctgcgccgccaggaggacttctaccccttcctgaaggacaaccgcgagaagatcgagaagatcctgaccttccgcatcccctactacgtgggccccctggcccgcggcaacagccgcttcgcctggatgacccgcaagagcgaggagaccatcaccccctggaacttcgaggaggtggtggacaagggcgccagcgcccagagcttcatcgagcgcatgaccaacttcgacaagaacctgcccaacgagaaggtgctgcccaagcacagcctgctgtacgagtacttcaccgtgtacaacgagctgaccaaggtgaagtacgtgaccgagggcatgcgcaagcccgccttcctgagcggcgagcagaagaaggccatcgtggacctgctgttcaagaccaaccgcaaggtgaccgtgaagcagctgaaggaggactacttcaagaagatcgagtgcttcgacagcgtggagatcagcggcgtggaggaccgcttcaacgccagcctgggcacctaccacgacctgctgaagatcatcaaggacaaggacttcctggacaacgaggagaacgaggacatcctggaggacatcgtgctgaccctgaccctgttcgaggaccgcgagatgatcgaggagcgcctgaagacctacgcccacctgttcgacgacaaggtgatgaagcagctgaagcgccgccgctacaccggctggggccgcctgagccgcaagcttatcaacggcatccgcgacaagcagagcggcaagaccatcctggacttcctgaagagcgacggcttcgccaaccgcaacttcatgcagctgatccacgacgacagcctgaccttcaaggaggacatccagaaggcccaggtgagcggccagggcgacagcctgcacgagcacatcgccaacctggccggcagccccgccatcaagaagggcatcctgcagaccgtgaaggtggtggacgagctggtgaaggtgatgggccgccacaagcccgagaacatcgtgatcgagatggcccgcgagaaccagaccacccagaagggccagaagaacagccgcgagcgcatgaagcgcatcgaggagggcatcaaggagctgggcagccagatcctgaaggagcaccccgtggagaacacccagctgcagaacgagaagctgtacctgtactacctgcagaacggccgcgacatgtacgtggaccaggagctggacatcaaccgcctgagcgactacgacgtggaccacatcgtgccccagagcttcctgaaggacgacagcatcgacaacaaggtgctgacccgcagcgacaagaaccgcggcaagagcgacaacgtgcccagcgaggaggtggtgaagaagatgaagaactactggcgccagctgctgaacgccaagctgatcacccagcgcaagttcgacaacctgaccaaggccgagcgcggcggcctgagcgagctggacaaggccggcttcatcaagcgccagctggtggagacccgccagatcaccaagcacgtggcccagatcctggacagccgcatgaacaccaagtacgacgagaacgacaagctgatccgcgaggtgaaggtgatcaccctgaagagcaagctggtgagcgacttccgcaaggacttccagttctacaaggtgcgcgagatcaacaactaccaccacgcccacgacgcctacctgaacgccgtggtgggcaccgccctgatcaagaagtaccccaagctggagagcgagttcgtgtacggcgactacaaggtgtacgacgtgcgcaagatgatcgccaagagcgagcaggagatcggcaaggccaccgccaagtacttcttctacagcaacatcatgaacttcttcaagaccgagatcaccctggccaacggcgagatccgcaagcgccccctgatcgagaccaacggcgagaccggcgagatcgtgtgggacaagggccgcgacttcgccaccgtgcgcaaggtgctgagcatgccccaggtgaacatcgtgaagaagaccgaggtgcagaccggcggcttcagcaaggagagcatcctgcccaagcgcaacagcgacaagctgatcgcccgcaagaaggactgggaccccaagaagtacggcggcttcgacagccccaccgtggcctacagcgtgctggtggtggccaaggtggagaagggcaagagcaagaagctgaagagcgtgaaggagctgctgggcatcaccatcatggagcgcagcagcttcgagaagaaccccatcgacttcctggaggccaagggctacaaggaggtgaagaaggacctgatcatcaagctgcccaagtacagcctgttcgagctggagaacggccgcaagcgcatgctggccagcgccggcgagctgcagaagggcaacgagctggccctgcccagcaagtacgtgaacttcctgtacctggccagccactacgagaagctgaagggcagccccgaggacaacgagcagaagcagctgttcgtggagcagcacaagcactacctggacgagatcatcgagcagatcagcgagttcagcaagcgcgtgatcctggccgacgccaacctggacaaggtgctgagcgcctacaacaagcaccgcgacaagcccatccgcgagcaggccgagaacatcatccacctgttcaccctgaccaacctgggcgcccccgccgccttcaagtacttcgacaccaccatcgaccgcaagcgctacaccagcaccaaggaggtgctggacgccaccctgatccaccagagcatcaccggtctgtacgagacccgcatcgacctgagccagctgggcggcgacggcggctccggacctccaaagaaaaagagaaaagtatacccctacgacgtgcccgactacgcctaa

SEQ ID NO: 107 - DNA, 4194 bp, synthetic construct
  misc_feature 1..4194: note = Description of Artificial Sequence: Synthetic polynucleotide
  misc_feature 1..4194: note = Cas9 coding sequence in p3s-Cas9HN (humanized codon, N-term tagging (underlined), human cell experiments)
  source 1..4194: mol_type = other DNA
atggtgtacccctacgacgtgcccgactacgccgaattgcctccaaaaaagaagagaaaggtagggatccgaattcccggggaaaaaccggacaagaagtacagcatcggcctggacatcggtaccaacagcgtgggctgggccgtgatcaccgacgagtacaaggtgcccagcaagaagttcaaggtgctgggcaacaccgaccgccacagcatcaagaagaacctgatcggcgccctgctgttcgacagcggcgagaccgccgaggccacccgcctgaagcgcaccgcccgccgccgctacacccgccgcaagaaccgcatctgctacctgcaggagatcttcagcaacgagatggccaaggtggacgacagcttcttccaccgcctggaggagagcttcctggtggaggaggacaagaagcacgagcgccaccccatcttcggcaacatcgtggacgaggtggcctaccacgagaagtaccccaccatctaccacctgcgcaagaagctggtggacagcaccgacaaggccgacctgcgcctgatctacctggccctggcccacatgatcaagttccgcggccacttcctgatcgagggcgacctgaaccccgacaacagcgacgtggacaagctgttcatccagctggtgcagacctacaaccagctgttcgaggagaaccccatcaacgccagcggcgtggacgccaaggccatcctgagcgcccgcctgagcaagagccgccgcctggagaacctgatcgcccagctgcccggcgagaagaagaacggcctgttcggcaacctgatcgccctgagcctgggcctgacccccaacttcaagagcaacttcgacctggccgaggacgccaagctgcagctgagcaaggacacctacgacgacgacctggacaacctgctggcccagatcggcgaccagtacgccgacctgttcctggccgccaagaacctgagcgacgccatcctgctgagcgacatcctgcgcgtgaacaccgagatcaccaaggcccccctgagcgccagcatgatcaagcgctacgacgagcaccaccaggacctgaccctgctgaaggccctggtgcgccagcagctgcccgagaagtacaaggagatcttcttcgaccagagcaagaacggctacgccggctacatcgacggcggcgccagccaggaggagttctacaagttcatcaagcccatcctggagaagatggacggcaccgaggagctgctggtgaagctgaaccgcgaggacctgctgcgcaagcagcgcaccttcgacaacggcagcatcccccaccagatccacctgggcgagctgcacgccatcctgcgccgccaggaggacttctaccccttcctgaaggacaaccgcgagaagatcgagaagatcctgaccttccgcatcccctactacgtgggccccctggcccgcggcaacagccgcttcgcctggatgacccgcaagagcgaggagaccatcaccccctggaacttcgaggaggtggtggacaagggcgccagcgcccagagcttcatcgagcgcatgaccaacttcgacaagaacctgcccaacgagaaggtgctgcccaagcacagcctgctgtacgagtacttcaccgtgtacaacgagctgaccaaggtgaagtacgtgaccgagggcatgcgcaagcccgccttcctgagcggcgagcagaagaaggccatcgtggacctgctgttcaagaccaaccgcaaggtgaccgtgaagcagctgaaggaggactacttcaagaagatcgagtgcttcgacagcgtggagatcagcggcgtggaggaccgcttcaacgccagcctgggcacctaccacgacctgctgaagatcatcaaggacaaggacttcctggacaacgaggagaacgaggacatcctggaggacatcgtgctgaccctgaccctgttcgaggaccgcgagatgatcgaggagcgcctgaagacctacgcccacctgttcgacgacaaggtgatgaagcagctgaagcgccgccgctacaccggctggggccgcctgagccgcaagcttatcaacggcatccgcgacaagcagagcggcaagaccatcctggacttcctgaagagcgacggcttcgccaaccgcaacttcatgcagctgatccacgacgacagcctgaccttcaaggaggacatccagaaggcccaggtgagcggccagggcgacagcctgcacgagcacatcgccaacctggccggcagccccgccatcaagaagggcatcctgcagaccgtgaaggtggtggacgagctggtgaaggtgatgggccgccacaagcccgagaacatcgtgatcgagatggcccgcgagaaccagaccacccagaagggccagaagaacagccgcgagcgcatgaagcgcatcgaggagggcatcaaggagctgggcagccagatcctgaaggagcaccccgtggagaacacccagctgcagaacgagaagctgtacctgtactacctgcagaacggccgcgacatgtacgtggaccaggagctggacatcaaccgcctgagcgactacgacgtggaccacatcgtgccccagagcttcctgaaggacgacagcatcgacaacaaggtgctgacccgcagcgacaagaaccgcggcaagagcgacaacgtgcccagcgaggaggtggtgaagaagatgaagaactactggcgccagctgctgaacgccaagctgatcacccagcgcaagttcgacaacctgaccaaggccgagcgcggcggcctgagcgagctggacaaggccggcttcatcaagcgccagctggtggagacccgccagatcaccaagcacgtggcccagatcctggacagccgcatgaacaccaagtacgacgagaacgacaagctgatccgcgaggtgaaggtgatcaccctgaagagcaagctggtgagcgacttccgcaaggacttccagttctacaaggtgcgcgagatcaacaactaccaccacgcccacgacgcctacctgaacgccgtggtgggcaccgccctgatcaagaagtaccccaagctggagagcgagttcgtgtacggcgactacaaggtgtacgacgtgcgcaagatgatcgccaagagcgagcaggagatcggcaaggccaccgccaagtacttcttctacagcaacatcatgaacttcttcaagaccgagatcaccctggccaacggcgagatccgcaagcgccccctgatcgagaccaacggcgagaccggcgagatcgtgtgggacaagggccgcgacttcgccaccgtgcgcaaggtgctgagcatgccccaggtgaacatcgtgaagaagaccgaggtgcagaccggcggcttcagcaaggagagcatcctgcccaagcgcaacagcgacaagctgatcgcccgcaagaaggactgggaccccaagaagtacggcggcttcgacagccccaccgtggcctacagcgtgctggtggtggccaaggtggagaagggcaagagcaagaagctgaagagcgtgaaggagctgctgggcatcaccatcatggagcgcagcagcttcgagaagaaccccatcgacttcctggaggccaagggctacaaggaggtgaagaaggacctgatcatcaagctgcccaagtacagcctgttcgagctggagaacggccgcaagcgcatgctggccagcgccggcgagctgcagaagggcaacgagctggccctgcccagcaagtacgtgaacttcctgtacctggccagccactacgagaagctgaagggcagccccgaggacaacgagcagaagcagctgttcgtggagcagcacaagcactacctggacgagatcatcgagcagatcagcgagttcagcaagcgcgtgatcctggccgacgccaacctggacaaggtgctgagcgcctacaacaagcaccgcgacaagcccatccgcgagcaggccgagaacatcatccacctgttcaccctgaccaacctgggcgcccccgccgccttcaagtacttcgacaccaccatcgaccgcaagcgctacaccagcaccaaggaggtgctggacgccaccctgatccaccagagcatcaccggtctgtacgagacccgcatcgacctgagccagctgggcggcgactaa

SEQ ID NO: 108 - DNA, 4107 bp, synthetic construct
  misc_feature 1..4107: note = Description of Artificial Sequence: Synthetic polynucleotide
  misc_feature 1..4107: note = Cas9-coding sequence in Streptococcus pyogenes
  source 1..4107: mol_type = other DNA
atggataagaaatactcaataggcttagatatcggcacaaatagcgtcggatgggcggtgatcactgatgaatataaggttccgtctaaaaagttcaaggttctgggaaatacagaccgccacagtatcaaaaaaaatcttataggggctcttttatttgacagtggagagacagcggaagcgactcgtctcaaacggacagctcgtagaaggtatacacgtcggaagaatcgtatttgttatctacaggagattttttcaaatgagatggcgaaagtagatgatagtttctttcatcgacttgaagagtcttttttggtggaagaagacaagaagcatgaacgtcatcctatttttggaaatatagtagatgaagttgcttatcatgagaaatatccaactatctatcatctgcgaaaaaaattggtagattctactgataaagcggatttgcgcttaatctatttggccttagcgcatatgattaagtttcgtggtcattttttgattgagggagatttaaatcctgataatagtgatgtggacaaactatttatccagttggtacaaacctacaatcaattatttgaagaaaaccctattaacgcaagtggagtagatgctaaagcgattctttctgcacgattgagtaaatcaagacgattagaaaatctcattgctcagctccccggtgagaagaaaaatggcttatttgggaatctcattgctttgtcattgggtttgacccctaattttaaatcaaattttgatttggcagaagatgctaaattacagctttcaaaagatacttacgatgatgatttagataatttattggcgcaaattggagatcaatatgctgatttgtttttggcagctaagaatttatcagatgctattttactttcagatatcctaagagtaaatactgaaataactaaggctcccctatcagcttcaatgattaaacgctacgatgaacatcatcaagacttgactcttttaaaagctttagttcgacaacaacttccagaaaagtataaagaaatcttttttgatcaatcaaaaaacggatatgcaggttatattgatgggggagctagccaagaagaattttataaatttatcaaaccaattttagaaaaaatggatggtactgaggaattattggtgaaactaaatcgtgaagatttgctgcgcaagcaacggacctttgacaacggctctattccccatcaaattcacttgggtgagctgcatgctattttgagaagacaagaagacttttatccatttttaaaagacaatcgtgagaagattgaaaaaatcttgacttttcgaattccttattatgttggtccattggcgcgtggcaatagtcgttttgcatggatgactcggaagtctgaagaaacaattaccccatggaattttgaagaagttgtcgataaaggtgcttcagctcaatcatttattgaacgcatgacaaactttgataaaaatcttccaaatgaaaaagtactaccaaaacatagtttgctttatgagtattttacggtttataacgaattgacaaaggtcaaatatgttactgaaggaatgcgaaaaccagcatttctttcaggtgaacagaagaaagccattgttgatttactcttcaaaacaaatcgaaaagtaaccgttaagcaattaaaagaagattatttcaaaaaaatagaatgttttgatagtgttgaaatttcaggagttgaagatagatttaatgcttcattaggtacctaccatgatttgctaaaaattattaaagataaagattttttggataatgaagaaaatgaagatatcttagaggatattgttttaacattgaccttatttgaagatagggagatgattgaggaaagacttaaaacatatgctcacctctttgatgataaggtgatgaaacagcttaaacgtcgccgttatactggttggggacgtttgtctcgaaaattgattaatggtattagggataagcaatctggcaaaacaatattagattttttgaaatcagatggttttgccaatcgcaattttatgcagctgatccatgatgatagtttgacatttaaagaagacattcaaaaagcacaagtgtctggacaaggcgatagtttacatgaacatattgcaaatttagctggtagccctgctattaaaaaaggtattttacagactgtaaaagttgttgatgaattggtcaaagtaatggggcggcataagccagaaaatatcgttattgaaatggcacgtgaaaatcagacaactcaaaagggccagaaaaattcgcgagagcgtatgaaacgaatcgaagaaggtatcaaagaattaggaagtcagattcttaaagagcatcctgttgaaaatactcaattgcaaaatgaaaagctctatctctattatctccaaaatggaagagacatgtatgtggaccaagaattagatattaatcgtttaagtgattatgatgtcgatcacattgttccacaaagtttccttaaagacgattcaatagacaataaggtcttaacgcgttctgataaaaatcgtggtaaatcggataacgttccaagtgaagaagtagtcaaaaagatgaaaaactattggagacaacttctaaacgccaagttaatcactcaacgtaagtttgataatttaacgaaagctgaacgtggaggtttgagtgaacttgataaagctggttttatcaaacgccaattggttgaaactcgccaaatcactaagcatgtggcacaaattttggatagtcgcatgaatactaaatacgatgaaaatgataaacttattcgagaggttaaagtgattaccttaaaatctaaattagtttctgacttccgaaaagatttccaattctataaagtacgtgagattaacaattaccatcatgcccatgatgcgtatctaaatgccgtcgttggaactgctttgattaagaaatatccaaaacttgaatcggagtttgtctatggtgattataaagtttatgatgttcgtaaaatgattgctaagtctgagcaagaaataggcaaagcaaccgcaaaatatttcttttactctaatatcatgaacttcttcaaaacagaaattacacttgcaaatggagagattcgcaaacgccctctaatcgaaactaatggggaaactggagaaattgtctgggataaagggcgagattttgccacagtgcgcaaagtattgtccatgccccaagtcaatattgtcaagaaaacagaagtacagacaggcggattctccaaggagtcaattttaccaaaaagaaattcggacaagcttattgctcgtaaaaaagactgggatccaaaaaaatatggtggttttgatagtccaacggtagcttattcagtcctagtggttgctaaggtggaaaaagggaaatcgaagaagttaaaatccgttaaagagttactagggatcacaattatggaaagaagttcctttgaaaaaaatccgattgactttttagaagctaaaggatataaggaagttaaaaaagacttaatcattaaactacctaaatatagtctttttgagttagaaaacggtcgtaaacggatgctggctagtgccggagaattacaaaaaggaaatgagctggctctgccaagcaaatatgtgaattttttatatttagctagtcattatgaaaagttgaagggtagtccagaagataacgaacaaaaacaattgtttgtggagcagcataagcattatttagatgagattattgagcaaatcagtgaattttctaagcgtgttattttagcagatgccaatttagataaagttcttagtgcatataacaaacatagagacaaaccaatacgtgaacaagcagaaaatattattcatttatttacgttgacgaatcttggagctcccgctgcttttaaatattttgatacaacaattgatcgtaaacgatatacgtctacaaaagaagttttagatgccactcttatccatcaatccatcactggtctttatgaaacacgcattgatttgagtcagctaggaggtgactaa

SEQ ID NO: 109 - protein, 1368 aa, synthetic construct [sequence omitted]

SEQ ID NO: 110 - DNA, 4221 bp, synthetic construct
  misc_feature 1..4221: note = Description of Artificial Sequence: Synthetic polynucleotide
  misc_feature 1..4221: note = Cas9-coding sequence in pET-Cas9N3T for the production of recombinant Cas9 protein in E. coli (humanized codon; hexa-His-tag and a nuclear localization signal at the N terminus)
  source 1..4221: mol_type = other DNA
atgggcagcagccatcatcatcatcatcatgtgtacccctacgacgtgcccgactacgccgaattgcctccaaaaaagaagagaaaggtagggatcgagaacctgtacttccagggcgacaagaagtacagcatcggcctggacatcggtaccaacagcgtgggctgggccgtgatcaccgacgagtacaaggtgcccagcaagaagttcaaggtgctgggcaacaccgaccgccacagcatcaagaagaacctgatcggcgccctgctgttcgacagcggcgagaccgccgaggccacccgcctgaagcgcaccgcccgccgccgctacacccgccgcaagaaccgcatctgctacctgcaggagatcttcagcaacgagatggccaaggtggacgacagcttcttccaccgcctggaggagagcttcctggtggaggaggacaagaagcacgagcgccaccccatcttcggcaacatcgtggacgaggtggcctaccacgagaagtaccccaccatctaccacctgcgcaagaagctggtggacagcaccgacaaggccgacctgcgcctgatctacctggccctggcccacatgatcaagttccgcggccacttcctgatcgagggcgacctgaaccccgacaacagcgacgtggacaagctgttcatccagctggtgcagacctacaaccagctgttcgaggagaaccccatcaacgccagcggcgtggacgccaaggccatcctgagcgcccgcctgagcaagagccgccgcctggagaacctgatcgcccagctgcccggcgagaagaagaacggcctgttcggcaacctgatcgccctgagcctgggcctgacccccaacttcaagagcaacttcgacctggccgaggacgccaagctgcagctgagcaaggacacctacgacgacgacctggacaacctgctggcccagatcggcgaccagtacgccgacctgttcctggccgccaagaacctgagcgacgccatcctgctgagcgacatcctgcgcgtgaacaccgagatcaccaaggcccccctgagcgccagcatgatcaagcgctacgacgagcaccaccaggacctgaccctgctgaaggccctggtgcgccagcagctgcccgagaagtacaaggagatcttcttcgaccagagcaagaacggctacgccggctacatcgacggcggcgccagccaggaggagttctacaagttcatcaagcccatcctggagaagatggacggcaccgaggagctgctggtgaagctgaaccgcgaggacctgctgcgcaagcagcgcaccttcgacaacggcagcatcccccaccagatccacctgggcgagctgcacgccatcctgcgccgccaggaggacttctaccccttcctgaaggacaaccgcgagaagatcgagaagatcctgaccttccgcatcccctactacgtgggccccctggcccgcggcaacagccgcttcgcctggatgacccgcaagagcgaggagaccatcaccccctggaacttcgaggaggtggtggacaagggcgccagcgcccagagcttcatcgagcgcatgaccaacttcgacaagaacctgcccaacgagaaggtgctgcccaagcacagcctgctgtacgagtacttcaccgtgtacaacgagctgaccaaggtgaagtacgtgaccgagggcatgcgcaagcccgccttcctgagcggcgagcagaagaaggccatcgtggacctgctgttcaagaccaaccgcaaggtgaccgtgaagcagctgaaggaggactacttcaagaagatcgagtgcttcgacagcgtggagatcagcggcgtggaggaccgcttcaacgccagcctgggcacctaccacgacctgctgaagatcatcaaggacaaggacttcctggacaacgaggagaacgaggacatcctggaggacatcgtgctgaccctgaccctgttcgaggaccgcgagatgatcgaggagcgcctgaagacctacgcccacctgttcgacgacaaggtgatgaagcagctgaagcgccgccgctacaccggctggggccgcctgagccgcaagcttatcaacggcatccgcgacaagcagagcggcaagaccatcctggacttcctgaagagcgacggcttcgccaaccgcaacttcatgcagctgatccacgacgacagcctgaccttcaaggaggacatccagaaggcccaggtgagcggccagggcgacagcctgcacgagcacatcgccaacctggccggcagccccgccatcaagaagggcatcctgcagaccgtgaaggtggtggacgagctggtgaaggtgatgggccgccacaagcccgagaacatcgtgatcgagatggcccgcgagaaccagaccacccagaagggccagaagaacagccgcgagcgcatgaagcgcatcgaggagggcatcaaggagctgggcagccagatcctgaaggagcaccccgtggagaacacccagctgcagaacgagaagctgtacctgtactacctgcagaacggccgcgacatgtacgtggaccaggagctggacatcaaccgcctgagcgactacgacgtggaccacatcgtgccccagagcttcctgaaggacgacagcatcgacaacaaggtgctgacccgcagcgacaagaaccgcggcaagagcgacaacgtgcccagcgaggaggtggtgaagaagatgaagaactactggcgccagctgctgaacgccaagctgatcacccagcgcaagttcgacaacctgaccaaggccgagcgcggcggcctgagcgagctggacaaggccggcttcatcaagcgccagctggtggagacccgccagatcaccaagcacgtggcccagatcctggacagccgcatgaacaccaagtacgacgagaacgacaagctgatccgcgaggtgaaggtgatcaccctgaagagcaagctggtgagcgacttccgcaaggacttccagttctacaaggtgcgcgagatcaacaactaccaccacgcccacgacgcctacctgaacgccgtggtgggcaccgccctgatcaagaagtaccccaagctggagagcgagttcgtgtacggcgactacaaggtgtacgacgtgcgcaagatgatcgccaagagcgagcaggagatcggcaaggccaccgccaagtacttcttctacagcaacatcatgaacttcttcaagaccgagatcaccctggccaacggcgagatccgcaagcgccccctgatcgagaccaacggcgagaccggcgagatcgtgtgggacaagggccgcgacttcgccaccgtgcgcaaggtgctgagcatgccccaggtgaacatcgtgaagaagaccgaggtgcagaccggcggcttcagcaaggagagcatcctgcccaagcgcaacagcgacaagctgatcgcccgcaagaaggactgggaccccaagaagtacggcggcttcgacagccccaccgtggcctacagcgtgctggtggtggccaaggtggagaagggcaagagcaagaagctgaagagcgtgaaggagctgctgggcatcaccatcatggagcgcagcagcttcgagaagaaccccatcgacttcctggaggccaagggctacaaggaggtgaagaaggacctgatcatcaagctgcccaagtacagcctgttcgagctggagaacggccgcaagcgcatgctggccagcgccggcgagctgcagaagggcaacgagctggccctgcccagcaagtacgtgaacttcctgtacctggccagccactacgagaagctgaagggcagccccgaggacaacgagcagaagcagctgttcgtggagcagcacaagcactacctggacgagatcatcgagcagatcagcgagttcagcaagcgcgtgatcctggccgacgccaacctggacaaggtgctgagcgcctacaacaagcaccgcgacaagcccatccgcgagcaggccgagaacatcatccacctgttcaccctgaccaacctgggcgcccccgccgccttcaagtacttcgacaccaccatcgaccgcaagcgctacaccagcaccaaggaggtgctggacgccaccctgatccaccagagcatcaccggtctgtacgagacccgcatcgacctgagccagctgggcggcgactaa

SEQ ID NO: 111 - protein, 1406 aa, synthetic construct
  REGION 1..1406: note = Description of Artificial Sequence: Synthetic polypeptide
  REGION 1..1406: note = Amino acid sequence of Cas9 (pET-Cas9N3T)
MGSSHHHHHHVYPYDVPDYAELPPKKKRKVGIENLYFQGDKKYSIGLDIGTNSVGWAVITDEYKVPSKKFKVLGNTDRHSIKKNLIGALLFDSGETAEATRLKRTARRRYTRRKNRICYLQEIFSNEMAKVDDSFFHRLEESFLVEEDKKHERHPIFGNIVDEVAYHEKYPTIYHLRKKLVDSTDKADLRLIYLALAHMIKFRGHFLIEGDLNPDNSDVDKLFIQLVQTYNQLFEENPINASGVDAKAILSARLSKSRRLENLIAQLPGEKKNGLFGNLIALSLGLTPNFKSNFDLAEDAKLQLSKDTYDDDLDNLLAQIGDQYADLFLAAKNLSDAILLSDILRVNTEITKAPLSASMIKRYDEHHQDLTLLKALVRQQLPEKYKEIFFDQSKNGYAGYIDGGASQEEFYKFIKPILEKMDGTEELLVKLNREDLLRKQRTFDNGSIPHQIHLGELHAILRRQEDFYPFLKDNREKIEKILTFRIPYYVGPLARGNSRFAWMTRKSEETITPWNFEEVVDKGASAQSFIERMTNFDKNLPNEKVLPKHSLLYEYFTVYNELTKVKYVTEGMRKPAFLSGEQKKAIVDLLFKTNRKVTVKQLKEDYFKKIECFDSVEISGVEDRFNASLGTYHDLLKIIKDKDFLDNEENEDILEDIVLTLTLFEDREMIEERLKTYAHLFDDKVMKQLKRRRYTGWGRLSRKLINGIRDKQSGKTILDFLKSDGFANRNFMQLIHDDSLTFKEDIQKAQVSGQGDSLHEHIANLAGSPAIKKGILQTVKVVDELVKVMGRHKPENIVIEMARENQTTQKGQKNSRERMKRIEEGIKELGSQILKEHPVENTQLQNEKLYLYYLQNGRDMYVDQELDINRLSDYDVDHIVPQSFLKDDSIDNKVLTRSDKNRGKSDNVPSEEVVKKMKNYWRQLLNAKLITQRKFDNLTKAERGGLSELDKAGFIKRQLVETRQITKHVAQILDSRMNTKYDENDKLIREVKVITLKSKLVSDFRKDFQFYKVREINNYHHAHDAYLNAVVGTALIKKYPKLESEFVYGDYKVYDVRKMIAKSEQEIGKATAKYFFYSNIMNFFKTEITLANGEIRKRPLIETNGETGEIVWDKGRDFATVRKVLSMPQVNIVKKTEVQTGGFSKESILPKRNSDKLIARKKDWDPKKYGGFDSPTVAYSVLVVAKVEKGKSKKLKSVKELLGITIMERSSFEKNPIDFLEAKGYKEVKKDLIIKLPKYSLFELENGRKRMLASAGELQKGNELALPSKYVNFLYLASHYEKLKGSPEDNEQKQLFVEQHKHYLDEIIEQISEFSKRVILADANLDKVLSAYNKHRDKPIREQAENIIHLFTLTNLGAPAAFKYFDTTIDRKRYTSTKEVLDATLIHQSITGLYETRIDLSQLGGD

SEQ ID NO: 112 - DNA, 34 bp, Homo sapiens
  source 1..34: mol_type = other DNA
caatctatgacatcaattattatacatcggagcc

SEQ ID NO: 113 - RNA, 64 nt, synthetic construct
  misc_feature 1..64: note = Description of Artificial Sequence: Synthetic oligonucleotide
  source 1..64: mol_type = other RNA
ggtgacatcaattattatacatgttttagagctagaaatagcaagttaaaataaggctagtccg

SEQ ID NO: 114 - DNA, 49 bp, synthetic construct
  misc_feature 1..49: note = Description of Artificial Sequence: Synthetic oligonucleotide
  source 1..49: mol_type = other DNA
caatctatgacatcaattattatacatcggagccctgccaaaaaatcaa

SEQ ID NO: 115 - DNA, 50 bp, synthetic construct
  misc_feature 1..50: note = Description of Artificial Sequence: Synthetic oligonucleotide
  source 1..50: mol_type = other DNA
caatctatgacatcaattattataacatcggagccctgccaaaaaatcaa

SEQ ID NO: 116 - DNA, 36 bp, synthetic construct
  misc_feature 1..36: note = Description of Artificial Sequence: Synthetic oligonucleotide
  source 1..36: mol_type = other DNA
caatctatgacatcaattattatgccaaaaaatcaa

SEQ ID NO: 117 - DNA, 35 bp, synthetic construct
  misc_feature 1..35: note = Description of Artificial Sequence: Synthetic oligonucleotide
  source 1..35: mol_type = other DNA
caatctatgacatcggagccctgccaaaaaatcaa

SEQ ID NO: 118 - DNA, 31 bp, synthetic construct
  misc_feature 1..31: note = Description of Artificial Sequence: Synthetic oligonucleotide
  source 1..31: mol_type = other DNA
caatctatgacatgccctgccaaaaaatcaa

SEQ ID NO: 119 - DNA, 30 bp, synthetic construct
  misc_feature 1..30: note = Description of Artificial Sequence: Synthetic oligonucleotide
  source 1..30: mol_type = other DNA
caatctatgacatcaattattataaatcaa

SEQ ID NO: 120 - DNA, 25 bp, synthetic construct
  misc_feature 1..25: note = Description of Artificial Sequence: Synthetic oligonucleotide
  source 1..25: mol_type = other DNA
caatctatgacatccaaaaaatcaa

SEQ ID NO: 121 - DNA, 19 bp, synthetic construct
  misc_feature 1..19: note = Description of Artificial Sequence: Synthetic oligonucleotide
  source 1..19: mol_type = other DNA
caatctatgacaaaatcaa

SEQ ID NO: 122 - DNA, 46 bp, Homo sapiens
  source 1..46: mol_type = other DNA
tatgtgcaatgaccactacatcctcaagggcagcaatcggagccag

SEQ ID NO: 123 - DNA, 47 bp, synthetic construct
  misc_feature 1..47: note = Description of Artificial Sequence: Synthetic oligonucleotide
  source 1..47: mol_type = other DNA
tatgtgcaatgaccactacatccttcaagggcagcaatcggagccag

SEQ ID NO: 124 - DNA, 48 bp, synthetic construct
  misc_feature 1..48: note = Description of Artificial Sequence: Synthetic oligonucleotide
  source 1..48: mol_type = other DNA
tatgtgcaatgaccactacatcctctcaagggcagcaatcggagccag

SEQ ID NO: 125 - DNA, 18 bp, synthetic construct
  misc_feature 1..18: note = Description of Artificial Sequence: Synthetic oligonucleotide
  source 1..18: mol_type = other DNA
tatgtgcaatggagccag

SEQ ID NO: 126 - DNA, 13 bp, synthetic construct
  misc_feature 1..13: note = Description of Artificial Sequence: Synthetic oligonucleotide
  source 1..13: mol_type = other DNA
tatgtgcaatgac

SEQ ID NO: 127 - DNA, 23 bp, Homo sapiens
  source 1..23: mol_type = other DNA
tgacatcaattattatacatcgg

SEQ ID NO: 128 - DNA, 23 bp, Homo sapiens
  source 1..23: mol_type = other DNA
tgacatcaattattatagatgga

SEQ ID NO: 129 - DNA, 23 bp, Homo sapiens
  source 1..23: mol_type = other DNA
tgacatcacttattatgcatggg

SEQ ID NO: 130 - DNA, 23 bp, Homo sapiens
  source 1..23: mol_type = other DNA
tgacataaattattctacatggg

SEQ ID NO: 131 - DNA, 23 bp, Homo sapiens
  source 1..23: mol_type = other DNA
tgaaatcaattatcatagatcgg

SEQ ID NO: 132 - DNA, 23 bp, Homo sapiens
  source 1..23: mol_type = other DNA
ccaggctccacccgactggaggg

SEQ ID NO: 133 - RNA, 106 nt, synthetic construct
  misc_feature 1..106: note = Description of Artificial Sequence: Synthetic polynucleotide
  source 1..106: mol_type = other RNA
ggccaggctccacccgactggagttttagagctagaaatagcaagttaaaataaggctagtccgttatcaacttgaaaaagtggcaccgagtcggtgctttttttt

SEQ ID NO: 134 - DNA, 53 bp, Homo sapiens
  source 1..53: mol_type = other DNA
acttccaggctccacccgactggagggcgaaccccaaggggacctcatgcagg

SEQ ID NO: 135 - DNA, 13 bp, synthetic construct
  misc_feature 1..13: note = Description of Artificial Sequence: Synthetic oligonucleotide
  source 1..13: mol_type = other DNA
acttccaggctcc

SEQ ID NO: 136 - DNA, 30 bp, synthetic construct
  misc_feature 1..30: note = Description of Artificial Sequence: Synthetic oligonucleotide
  source 1..30: mol_type = other DNA
acttccaggctccacccgacctcatgcagg

SEQ ID NO: 137 - DNA, 36 bp, synthetic construct
  misc_feature 1..36: note = Description of Artificial Sequence: Synthetic oligonucleotide
  source 1..36: mol_type = other DNA
acttccaggctccaccccaaggggacctcatgcagg

SEQ ID NO: 138 - DNA, 54 bp, synthetic construct
  misc_feature 1..54: note = Description of Artificial Sequence: Synthetic oligonucleotide
  source 1..54: mol_type = other DNA
acttccaggctccacccgacttggagggcgaaccccaaggggacctcatgcagg

SEQ ID NO: 139 - DNA, 43 bp, synthetic construct
  misc_feature 1..43: note = Description of Artificial Sequence: Synthetic oligonucleotide
  source 1..43: mol_type = other DNA
acttccaggctccacccgaaccccaaggggacctcatgcaggg

SEQ ID NO: 140 - DNA, 47 bp, synthetic construct
  misc_feature 1..47: note = Description of Artificial Sequence: Synthetic oligonucleotide
  source 1..47: mol_type = other DNA
acttccaggctccacccgactcactatcttctgggctcctccatgtc

SEQ ID NO: 141 - DNA, 45 bp, synthetic construct
  misc_feature 1..45: note = Description of Artificial Sequence: Synthetic oligonucleotide
  source 1..45: mol_type = other DNA
acttccaggctccacccgacgaaccccaaggggacctcatgcagg

SEQ ID NO: 142 - protein, 18 aa, Homo sapiens
LPGSTRLEGEPQGDLMQA

SEQ ID NO: 143 - DNA, 57 bp, Homo sapiens
  source 1..57: mol_type = other DNA
  CDS 2..55
acttccaggctccacccgactggagggcgaaccccaaggggacctcatgcaggctcc

SEQ ID NO: 144 - DNA, 46 bp, synthetic construct
  misc_feature 1..46: note = Description of Artificial Sequence: Synthetic oligonucleotide
  source 1..46: mol_type = other DNA
acttccaggctccacccgaaccccaaggggacctcatgcaggctcc

SEQ ID NO: 145 - DNA, 43 bp, synthetic construct
  misc_feature 1..43: note = Description of Artificial Sequence: Synthetic oligonucleotide
  source 1..43: mol_type = other DNA
acttccaggctccacccgaaccccaaggggacctcatgcaggc

SEQ ID NO: 146 - DNA, 20 bp, synthetic construct
  misc_feature 1..20: note = Description of Artificial Sequence: Synthetic oligonucleotide
  source 1..20: mol_type = other DNA
acttccaggctccacccgac

SEQ ID NO: 147 - DNA, 40 bp, synthetic construct
  misc_feature 1..40: note = Description of Artificial Sequence: Synthetic oligonucleotide
  source 1..40: mol_type = other DNA
acttccaggctccaccccaaggggacctcatgcaggctcc

SEQ ID NO: 148 - DNA, 58 bp, synthetic construct
  misc_feature 1..58: note = Description of Artificial Sequence: Synthetic oligonucleotide
  source 1..58: mol_type = other DNA
acttccaggctccacccgacttggagggcgaaccccaaggggacctcatgcaggctcc

SEQ ID NO: 149 - DNA, 46 bp, synthetic construct
  misc_feature 1..46: note = Description of Artificial Sequence: Synthetic oligonucleotide
  source 1..46: mol_type = other DNA
acttccaggctccaggcgaaccccaaggggacctcatgcaggctcc

SEQ ID NO: 150 - DNA, 32 bp, synthetic construct
  misc_feature 1..32: note = Description of Artificial Sequence: Synthetic oligonucleotide
  source 1..32: mol_type = other DNA
ggcgaaccccaaggggacctcatgcaggctcc

SEQ ID NO: 151 - DNA, 32 bp, synthetic construct
  misc_feature 1..32: note = Description of Artificial Sequence: Synthetic oligonucleotide
  source 1..32: mol_type = other DNA
acttccaggcaaggggacctcatgcaggctcc

SEQ ID NO: 152 - DNA, 33 bp, synthetic construct
  misc_feature 1..33: note = Description of Artificial Sequence: Synthetic oligonucleotide
  source 1..33: mol_type = other DNA
acttccaggctaaggggacctcatgcaggctcc

SEQ ID NO: 153 - DNA, 52 bp, Homo sapiens
  source 1..52: mol_type = other DNA
acttccaggctccacccgactggagggcgaaccccaaggggacctcatgcag

SEQ ID NO: 154 - DNA, 34 bp, synthetic construct
  misc_feature 1..34: note = Description of Artificial Sequence: Synthetic oligonucleotide
  source 1..34: mol_type = other DNA
acttccaggcgaaccccaaggggacctcatgcag

SEQ ID NO: 155 - DNA, 32 bp, synthetic construct
  misc_feature 1..32: note = Description of Artificial Sequence: Synthetic oligonucleotide
  source 1..32: mol_type = other DNA
acttccaggctccacaaggggacctcatgcag

SEQ ID NO: 156 - DNA, 34 bp, synthetic construct
  misc_feature 1..34: note = Description of Artificial Sequence: Synthetic oligonucleotide
  source 1..34: mol_type = other DNA
acttccaggctccacccaaggggacctcatgccc

SEQ ID NO: 157 - DNA, 35 bp, synthetic construct
  misc_feature 1..35: note = Description of Artificial Sequence: Synthetic oligonucleotide
  source 1..35: mol_type = other DNA
acttccaggctccaccccaaggggacctcatgcag

SEQ ID NO: 158 - DNA, 41 bp, synthetic construct
  misc_feature 1..41: note = Description of Artificial Sequence: Synthetic oligonucleotide
  source 1..41: mol_type = other DNA
acttccaggctccacccgaaccccaaggggacctcatgcag

SEQ ID NO: 159 - DNA, 50 bp, synthetic construct
  misc_feature 1..50: note = Description of Artificial Sequence: Synthetic oligonucleotide
  source 1..50: mol_type = other DNA
acttccaggctccacccgaaggagggcgaaccccaaggggacctcatgca

SEQ ID NO: 160 - DNA, 50 bp, synthetic construct
  misc_feature 1..50: note = Description of Artificial Sequence: Synthetic oligonucleotide
  source 1..50: mol_type = other DNA
acttccaggctccacccgactagggcgaaccccaaggggacctcatgcag

SEQ ID NO: 161 - DNA, 52 bp, synthetic construct
  misc_feature 1..52: note = Description of Artificial Sequence: Synthetic oligonucleotide
  source 1..52: mol_type = other DNA
acttccaggctccacccgactgggagggcgaaccccaaggggacctcatgca

SEQ ID NO: 162 - DNA, 52 bp, synthetic construct
  misc_feature 1..52: note = Description of Artificial Sequence: Synthetic oligonucleotide
  source 1..52: mol_type = other DNA
acttccaggctccacccgacttggagggcgaaccccaaggggacctcatgca

SEQ ID NO: 163 - DNA, 46 bp, synthetic construct
  misc_feature 1..46: note = Description of Artificial Sequence: Synthetic oligonucleotide
  source 1..46: mol_type = other DNA
acttccaggctccacccgaggcgaaccccaaggggacctcatgcag

SEQ ID NO: 164 - DNA, 47 bp, synthetic construct
  misc_feature 1..47: note = Description of Artificial Sequence: Synthetic oligonucleotide
  source 1..47: mol_type = other DNA
acttccaggctccacccgagggcgaaccccaaggggacctcatgcag

SEQ ID NO: 165 - DNA, 24 bp, synthetic construct
  misc_feature 1..24: note = Description of Artificial Sequence: Synthetic oligonucleotide
  source 1..24: mol_type = other DNA
acttccaggctccacctcatgcag

SEQ ID NO: 166 - DNA, 29 bp, synthetic construct
  misc_feature 1..29: note = Description of Artificial Sequence: Synthetic oligonucleotide
  source 1..29: mol_type = other DNA
agggcgaaccccaaggggacctcatgcag

SEQ ID NO: 167 - DNA, 45 bp, synthetic construct
  misc_feature 1..45: note = Description of Artificial Sequence: Synthetic oligonucleotide
  source 1..45: mol_type = other DNA
caatctatgacatcaattattatcggagccctgccaaaaaatcaa

SEQ ID NO: 168 - DNA, 45 bp, synthetic construct
  misc_feature 1..45: note = Description of Artificial Sequence: Synthetic oligonucleotide
  source 1..45: mol_type = other DNA
caatctatgacatcaattatcatcggagccctgccaaaaaatcaa

SEQ ID NO: 169 - DNA, 42 bp, synthetic construct
  misc_feature 1..42: note = Description of Artificial Sequence: Synthetic oligonucleotide
  source 1..42: mol_type = other DNA
caatctatgacatcaattatcggagccctgccaaaaaatcaa

SEQ ID NO: 170 - DNA, 48 bp, synthetic construct
  misc_feature 1..48: note = Description of Artificial Sequence: Synthetic oligonucleotide
  source 1..48: mol_type = other DNA
caatctatgacatcaattattatcatcggagccctgccaaaaaatcaa

SEQ ID NO: 171 - DNA, 33 bp, synthetic construct
  misc_feature 1..33: note = Description of Artificial Sequence: Synthetic oligonucleotide
  source 1..33: mol_type = other DNA
caatctatgacaagagccctgccaaaaaatcaa

SEQ ID NO: 172 - DNA, 52 bp, Homo sapiens
  source 1..52: mol_type = other DNA
ttctcaaggcagcatcatacttcccccacggtgggacagctgccctccctgg

SEQ ID NO: 173 - DNA, 46 bp, synthetic construct
  misc_feature 1..46: note = Description of Artificial Sequence: Synthetic oligonucleotide
  source 1..46: mol_type = other DNA
ttctcaaggcagcatcatacttccctgggacagctgccctccctgg

SEQ ID NO: 174 - DNA, 49 bp, synthetic construct
  misc_feature 1..49: note = Description of Artificial Sequence: Synthetic oligonucleotide
  source 1..49: mol_type = other DNA
ttctcaaggcagcatcatacttccacggtgggacagctgccctccctgg

SEQ ID NO: 175 - DNA, 25 bp, synthetic construct
  misc_feature 1..25: note = Description of Artificial Sequence: Synthetic oligonucleotide
  source 1..25: mol_type = other DNA
ttctcaaggcagctgccctccctgg

SEQ ID NO: 176 - DNA, 32 bp, synthetic construct
  misc_feature 1..32: note = Description of Artificial Sequence: Synthetic oligonucleotide
  source 1..32: mol_type = other DNA
ttctcaaggcagcatcatacttccctccctgg

SEQ ID NO: 177 - DNA, 264 bp, Homo sapiens
  modified_base 38..227: mod_base = OTHER; note = a, c, t, g, or unknown
  source 1..264: mol_type = other DNA
acaaagcgattttgaaagatggaagcgcggtggctatnnnnnnnnnnnnnnnnnnnnnnnnnnnnnnnnnnnnnnnnnnnnnnnnnnnnnnnnnnnnnnnnnnnnnnnnnnnnnnnnnnnnnnnnnnnnnnnnnnnnnnnnnnnnnnnnnnnnnnnnnnnnnnnnnnnnnnnnnnnnnnnnnnnnnnnnnnnnnnnnnnnnnnnnnnnnnnnnnnnnnnnnnnnnnnggggtgaaactaaactggtccacacggcggaagattg

SEQ ID NO: 178 - DNA, 257 bp, synthetic construct
  misc_feature 1..257: note = Description of Artificial Sequence: Synthetic polynucleotide
  modified_base 38..227: mod_base = OTHER; note = a, c, t, g, or unknown
  source 1..257: mol_type = other DNA
acaaagcgattttgaaagatggaagcgcggtggctatnnnnnnnnnnnnnnnnnnnnnnnnnnnnnnnnnnnnnnnnnnnnnnnnnnnnnnnnnnnnnnnnnnnnnnnnnnnnnnnnnnnnnnnnnnnnnnnnnnnnnnnnnnnnnnnnnnnnnnnnnnnnnnnnnnnnnnnnnnnnnnnnnnnnnnnnnnnnnnnnnnnnnnnnnnnnnnnnnnnnnnnnnnnnnnggggtgaaactaaaacacggcggaagattg

SEQ ID NO: 179 - DNA, 43 bp, synthetic construct
  misc_feature 1..43: note = Description of Artificial Sequence: Synthetic oligonucleotide
  source 1..43: mol_type = other DNA
acaaagcgattttgaaagatggaagcgacacggcggaagattg

SEQ ID NO: 180 - DNA, 44 bp, synthetic construct
  misc_feature 1..44: note = Description of Artificial Sequence: Synthetic oligonucleotide
  source 1..44: mol_type = other DNA
acaaagcgattttgaaagatggaagcgcacacggcggaagattg

SEQ ID NO: 181 - DNA, 106 bp, synthetic construct
  misc_feature 1..106: note = Description of Artificial Sequence: Synthetic polynucleotide
  source 1..106: mol_type = other DNA
acaaagcgattttgaaagatggaagcgaaatagcaagttaaaataaggctagtccgttatcaacttgaaaaagtggcaccgagtcggtgcacacggcggaagattg

SEQ ID NO: 182 - DNA, 23 bp, synthetic construct
  misc_feature 1..23: note = Description of Artificial Sequence: Synthetic oligonucleotide
  source 1..23: mol_type = other DNA
gggtggggggagtttgctcctgg

SEQ ID NO: 183 - DNA, 23 bp, synthetic construct
  misc_feature 1..23: note = Description of Artificial Sequence: Synthetic oligonucleotide
  source 1..23: mol_type = other DNA
ggatggagggagtttgctcctgg

SEQ ID NO: 184 - DNA, 23 bp, synthetic construct
  misc_feature 1..23: note = Description of Artificial Sequence: Synthetic oligonucleotide
  source 1..23: mol_type = other DNA
ggggaggggaagtttgctcctgg

SEQ ID NO: 185 - DNA, 23 bp, synthetic construct
  misc_feature 1..23: note = Description of Artificial Sequence: Synthetic oligonucleotide
  source 1..23: mol_type = other DNA
gaccccctccaccccgcctccgg

SEQ ID NO: 186 - DNA, 23 bp, synthetic construct
  misc_feature 1..23: note = Description of Artificial Sequence: Synthetic oligonucleotide
  source 1..23: mol_type = other DNA
gaccccccccaccccgcccccgg

SEQ ID NO: 187 - DNA, 23 bp, synthetic construct
  misc_feature 1..23: note = Description of Artificial Sequence: Synthetic oligonucleotide
  source 1..23: mol_type = other DNA
gcccccacccaccccgcctctgg

SEQ ID NO: 188 - DNA, 23 bp, synthetic construct
  misc_feature 1..23: note = Description of Artificial Sequence: Synthetic oligonucleotide
  source 1..23: mol_type = other DNA
ctccccacccaccccgcctcagg

SEQ ID NO: 189 - DNA, 23 bp, synthetic construct
  misc_feature 1..23: note = Description of Artificial Sequence: Synthetic oligonucleotide
  source 1..23: mol_type = other DNA
ggtgagtgagtgtgtgcgtgtgg

SEQ ID NO: 190 - DNA, 23 bp, synthetic construct
  misc_feature 1..23: note = Description of Artificial Sequence: Synthetic oligonucleotide
  source 1..23: mol_type = other DNA
tgtgggtgagtgtgtgcgtgagg

SEQ ID NO: 191 - DNA, 23 bp, synthetic construct
  misc_feature 1..23: note = Description of Artificial Sequence: Synthetic oligonucleotide
  source 1..23: mol_type = other DNA
gagtccgagcagaagaagaaggg

SEQ ID NO: 192 - DNA, 23 bp, synthetic construct
  misc_feature 1..23: note = Description of Artificial Sequence: Synthetic oligonucleotide
  source 1..23: mol_type = other DNA
gagttagagcagaagaagaaagg

SEQ ID NO: 193 - DNA, 23 bp, synthetic construct
  misc_feature 1..23: note = Description of Artificial Sequence: Synthetic oligonucleotide
  source 1..23: mol_type = other DNA
gaacctgagctgctctgacgcgg

SEQ ID NO: 194 - DNA, 23 bp, synthetic construct
  misc_feature 1..23: note = Description of Artificial Sequence: Synthetic oligonucleotide
  source 1..23: mol_type = other DNA
ttggcagggggtgggagggaagg

SEQ ID NO: 195 - DNA, 23 bp, synthetic construct
  misc_feature 1..23: note = Description of Artificial Sequence: Synthetic oligonucleotide
  source 1..23: mol_type = other DNA
gggagggagagcttggcaggggg

SEQ ID NO: 196 - DNA, 23 bp, synthetic construct
  misc_feature 1..23: note = Description of Artificial Sequence: Synthetic oligonucleotide
  source 1..23: mol_type = other DNA
gatggagccagagaggatcctgg

SEQ ID NO: 197 - DNA, 23 bp, synthetic construct
  misc_feature 1..23: note = Description of Artificial Sequence: Synthetic oligonucleotide
  source 1..23: mol_type = other DNA
cctgccaagctctccctcccagg

SEQ ID NO: 198 - DNA, 23 bp, synthetic construct
  misc_feature 1..23: note = Description of Artificial Sequence: Synthetic oligonucleotide
  source 1..23: mol_type = other DNA
ctccctcccaggatcctctctgg

SEQ ID NO: 199 - DNA, 23 bp, synthetic construct
  misc_feature 1..23: note = Description of Artificial Sequence: Synthetic oligonucleotide
  source 1..23: mol_type = other DNA
cctctaaggtttgcttacgatgg

SEQ ID NO: 200 - DNA, 23 bp, synthetic construct
  misc_feature 1..23: note = Description of Artificial Sequence: Synthetic oligonucleotide
  source 1..23: mol_type = other DNA
ggttctggcaaggagagagatgg

SEQ ID NO: 201 - DNA, 23 bp, synthetic construct
  misc_feature 1..23: note = Description of Artificial Sequence: Synthetic oligonucleotide
  source 1..23: mol_type = other DNA
tctaacccccacctcctgttagg

SEQ ID NO: 202 - DNA, 23 bp, synthetic construct
  misc_feature 1..23: note = Description of Artificial Sequence: Synthetic oligonucleotide
  source 1..23: mol_type = other DNA
ttggcagggggtgggagggatgg

SEQ ID NO: 203 - DNA, 23 bp, synthetic construct
  misc_feature 1..23: note = Description of Artificial Sequence: Synthetic oligonucleotide
  source 1..23: mol_type = other DNA
ttggtagggggtgggagggatgg

SEQ ID NO: 204 - DNA, 23 bp, synthetic construct
  misc_feature 1..23: note = Description of Artificial Sequence: Synthetic oligonucleotide
  source 1..23: mol_type = other DNA
gggaaggggagcttggcaggtgg

SEQ ID NO: 205 - DNA, 23 bp, synthetic construct
  misc_feature 1..23: note = Description of Artificial Sequence: Synthetic oligonucleotide
  source 1..23: mol_type = other DNA
ggtagtgagagcttggcaggtgg

SEQ ID NO: 206 - DNA, 23 bp, synthetic construct
  misc_feature 1..23: note = Description of Artificial Sequence: Synthetic oligonucleotide
  source 1..23: mol_type = other DNA
ctccctcccaggatcctcccagg

SEQ ID NO: 207 - DNA, 23 bp, synthetic construct
  misc_feature 1..23: note = Description of Artificial Sequence: Synthetic oligonucleotide
  source 1..23: mol_type = other DNA
gtccatggcaggatcctctcagg

SEQ ID NO: 208 - DNA, 23 bp, synthetic construct
  misc_feature 1..23: note = Description of Artificial Sequence: Synthetic oligonucleotide
  source 1..23: mol_type = other DNA
ctcccccccagtatcctctcagg

SEQ ID NO: 209 - DNA, 108 bp, Homo sapiens
  source 1..108: mol_type = other DNA
ccaatctatgacatcaattattatacatcggagccctgccaaaaaatcaatgtgaagcaaatcgcagcccgcctcctgcctccgctctactcactggtgttcatcttt

SEQ ID NO: 210 - DNA, 138 bp, Homo sapiens
  source 1..138: mol_type = other DNA
ccaccctataattctgaacctgcagaagaatctgaacataaaaacaacaattacgaaccaaacctatttaaaactccacaaaggaaaccatcttataatcagctggcttcaactccaataatattcaaagagcaaggg

SEQ ID NO: 211 - DNA, 121 bp, Homo sapiens
  misc_feature 49..50: note = Nucleotides at these positions are non-consecutive and are separated by a non-disclosed sequence
  source 1..121: mol_type = other DNA
ggccgggaatcaagagtcacccagagacagtgaccaaccatccctgtttagctctccctcccaggatcctctctggctccatcgtaagcaaaccttagaggttctggcaaggagagagatg

SEQ ID NO: 212 - DNA, 77 bp, synthetic construct
  misc_feature 1..77: note = Description of Artificial Sequence: Synthetic oligonucleotide
  source 1..77: mol_type = other DNA
ggccgggaatcaagagtcacccagtgaccaaccatccctgtaagcaaaccttagaggttctggcaaggagagagatg

SEQ ID NO: 213 - DNA, 27 bp, synthetic construct
  misc_feature 1..27: note = Description of Artificial Sequence: Synthetic oligonucleotide
  source 1..27: mol_type = other DNA
ggccgggaatcaagagtcacccaggaa

SEQ ID NO: 214 - DNA, 79 bp, synthetic construct
  misc_feature 1..79: note = Description of Artificial Sequence: Synthetic oligonucleotide
  source 1..79: mol_type = other DNA
ggccgggaatcaagagtcacccagacctctctggctccatcgtaagcaaaccttagaggttctggcaaggagagagatg

SEQ ID NO: 215 - DNA, 28 bp, synthetic construct
  misc_feature 1..28: note = Description of Artificial Sequence: Synthetic oligonucleotide
  source 1..28: mol_type = other DNA
ggccgggaatcaagagtcaccctaacag

SEQ ID NO: 216 - DNA, 66 bp, synthetic construct
  misc_feature 1..66: note = Description of Artificial Sequence: Synthetic oligonucleotide
  source 1..66: mol_type = other DNA
ggccgggaatcaagacgctggctccatcgtaagcaaaccttagaggttctggcaaggagagagatg

SEQ ID NO: 217 - DNA, 47 bp, synthetic construct
  misc_feature 1..47: note = Description of Artificial Sequence: Synthetic oligonucleotide
  source 1..47: mol_type = other DNA
ggctccatcgtaagcaaaccttagaggttctggcaaggagagagatg

SEQ ID NO: 218 - DNA, 78 bp, synthetic construct
  misc_feature 1..78: note = Description of Artificial Sequence: Synthetic oligonucleotide
  source 1..78: mol_type = other DNA
ggccgggaatcaagagtcacccagactctctggctccatcgtaagcaaaccttagaggttctggcaaggagagagatg

SEQ ID NO: 219 - DNA, 80 bp, synthetic construct
  misc_feature 1..80: note = Description of Artificial Sequence: Synthetic oligonucleotide
  source 1..80: mol_type = other DNA
ggccgggaatcaagagtcacccagagacagtgaccaaccatcgtaagcaaaccttagaggttctggcaaggagagagatg

SEQ ID NO: 220 - DNA, 46 bp, synthetic construct
  misc_feature 1..46: note = Description of Artificial Sequence: Synthetic oligonucleotide
  source 1..46: mol_type = other DNA
ggtccatcgtaagcaaaccttagaggttctggcaaggagagagatg

SEQ ID NO: 221 - DNA, 69 bp, synthetic construct
  misc_feature 1..69: note = Description of Artificial Sequence: Synthetic oligonucleotide
  source 1..69: mol_type = other DNA
ggccgggaatcaagagtcacccatctccatcgtaagcaaaccttagaggttctggcaaggagagagatg

SEQ ID NO: 222 - DNA, 76 bp, synthetic construct
  misc_feature 1..76: note = Description of Artificial Sequence: Synthetic oligonucleotide
  source 1..76: mol_type = other DNA
ggccgggaatcaagagtcacccagactctggctccatcgtaagcaaaccttagaggttctggcaaggagagagatg

SEQ ID NO: 223 - DNA, 50 bp, synthetic construct
  misc_feature 1..50: note = Description of Artificial Sequence: Synthetic oligonucleotide
  source 1..50: mol_type = other DNA
ggccgggaatcaagagtcacccagagacagtgaccaaccatcccatatca

SEQ ID NO: 224 - DNA, 59 bp, synthetic construct
  misc_feature 1..59: note = Description of Artificial Sequence: Synthetic oligonucleotide
  source 1..59: mol_type = other DNA
ggccgggaatcaagagtcatcgtaagcaaaccttagaggttctggcaaggagagagatg

SEQ ID NO: 225 - DNA, 24 bp, synthetic construct
  misc_feature 1..24: note = Description of Artificial Sequence: Synthetic oligonucleotide
  source 1..24: mol_type = other DNA
aatgaccactacatccttcaaggg

SEQ ID NO: 226 - DNA, 25 bp, synthetic construct
  misc_feature 1..25: note = Description of Artificial Sequence: Synthetic oligonucleotide
  source 1..25: mol_type = other DNA
aatgaccactacatcctttcaaggg

SEQ ID NO: 227 - DNA, 26 bp, synthetic construct
  misc_feature 1..26: note = Description of Artificial Sequence: Synthetic oligonucleotide
  source 1..26: mol_type = other DNA
aatgaccactacatccttttcaaggg

SEQ ID NO: 228 - DNA, 22 bp, synthetic construct
  misc_feature 1..22: note = Description of Artificial Sequence: Synthetic oligonucleotide
  source 1..22: mol_type = other DNA
aatgaccactacatcctaaggg

SEQ ID NO: 229 - DNA, 21 bp, synthetic construct
  misc_feature 1..21: note = Description of Artificial Sequence: Synthetic oligonucleotide
  source 1..21: mol_type = other DNA
aatgaccactacatcctaggg

SEQ ID NO: 230 - DNA, 20 bp, synthetic construct
  misc_feature 1..20: note = Description of Artificial Sequence: Synthetic oligonucleotide
  source 1..20: mol_type = other DNA
aatgaccactacatcctggg

SEQ ID NO: 231 - DNA, 42 bp, Homo sapiens
  source 1..42: mol_type = other DNA
tatgtgcaatgaccactacatcctcaagggcagcaatcggag

SEQ ID NO: 232 - DNA, 45 bp, synthetic construct
  misc_feature 1..45: note = Description of Artificial Sequence: Synthetic oligonucleotide
  source 1..45: mol_type = other DNA
tatgtgcaatgaccactacatcctcctcaagggcagcaatcggag

SEQ ID NO: 233 - DNA, 30 bp, synthetic construct
  misc_feature 1..30: note = Description of Artificial Sequence: Synthetic oligonucleotide
  source 1..30: mol_type = other DNA
tatgtgcaatgaccactacatcaatcggag

SEQ ID NO: 234 - DNA, 33 bp, synthetic construct
  misc_feature 1..33: note = Description of Artificial Sequence: Synthetic oligonucleotide
  source 1..33: mol_type = other DNA
tatgtgcaatgaccactacatcagcaatcggag

SEQ ID NO: 235 - DNA, 34 bp, synthetic construct
  misc_feature 1..34: note = Description of Artificial Sequence: Synthetic oligonucleotide
  source 1..34: mol_type = other DNA
tatgtgcaatgaccactacatccagcaatcggag

SEQ ID NO: 236 - DNA, 10 bp, synthetic construct
  misc_feature 1..10: note = Description of Artificial Sequence: Synthetic oligonucleotide
  source 1..10: mol_type = other DNA
cagcaatcgg

SEQ ID NO: 237 - DNA, 41 bp, synthetic construct
  misc_feature 1..41: note = Description of Artificial Sequence: Synthetic oligonucleotide
  source 1..41: mol_type = other DNA
tatgtgcaatgaccactacatccttcaagggcagcaatcgg

SEQ ID NO: 238 - DNA, 41 bp, synthetic construct
  misc_feature 1..41: note = Description of Artificial Sequence: Synthetic oligonucleotide
  source 1..41: mol_type = other DNA
tatgtgcaatgaccactacatcctccaagggcagcaatcgg

SEQ ID NO: 239 - DNA, 41 bp, synthetic construct
  misc_feature 1..41: note = Description of Artificial Sequence: Synthetic oligonucleotide
  source 1..41: mol_type = other DNA
tatgtgcaatgaccactacatcctbcaagggcagcaatcgg

SEQ ID NO: 240 - DNA, 34 bp, synthetic construct
  misc_feature 1..34: note = Description of Artificial Sequence: Synthetic oligonucleotide
  source 1..34: mol_type = other DNA
tatgtgcaatgaccactacattggcagcaatcgg

SEQ ID NO: 241 - DNA, 21 bp, synthetic construct
  misc_feature 1..21: note = Description of Artificial Sequence: Synthetic oligonucleotide
  source 1..21: mol_type = other DNA
tatgtgcaatgaccactacat

SEQ ID NO: 242 - DNA, 53 bp, Homo sapiens
  source 1..53: mol_type = other DNA
tcatacagatgatgtctcatcatcagaggagcgagaaggtaaagtcaaaatca

SEQ ID NO: 243 - DNA, 32 bp, synthetic construct
  misc_feature 1..32: note = Description of Artificial Sequence: Synthetic oligonucleotide
  source 1..32: mol_type = other DNA
tcatacagatgatacaggtaaagtcaaaatca

SEQ ID NO: 244 - DNA, 32 bp, synthetic construct
  misc_feature 1..32: note = Description of Artificial Sequence: Synthetic oligonucleotide
  source 1..32: mol_type = other DNA
tcatacaggtgatgaaggtaaagtcaaaatca

SEQ ID NO: 245 - DNA, 50 bp, synthetic construct
  misc_feature 1..50: note = Description of Artificial Sequence: Synthetic oligonucleotide
  source 1..50: mol_type = other DNA
tcatacagatgatgtctcatcatcagagcgagaaggtaaagtcaaaatca

SEQ ID NO: 246 - DNA, 48 bp, synthetic construct
  misc_feature 1..48: note = Description of Artificial Sequence: Synthetic oligonucleotide
  source 1..48: mol_type = other DNA
tcatacagatgatgtctcatcatcagcgagaaggtaaagtcaaaatca

SEQ ID NO: 247 - DNA, 52 bp, synthetic construct
  misc_feature 1..52: note = Description of Artificial Sequence: Synthetic oligonucleotide
  source 1..52: mol_type = other DNA
tcatacagatgatgtctcatcatcagggagcgagaaggtaaagtcaaaatca

SEQ ID NO: 248 - DNA, 41 bp, synthetic construct
  misc_feature 1..41: note = Description of Artificial Sequence: Synthetic oligonucleotide
  source 1..41: mol_type = other DNA
tcatacagatgatgtctcgcgagaaggtaaagtcaaaatca

SEQ ID NO: 249 - DNA, 32 bp, synthetic construct
  misc_feature 1..32: note = Description of Artificial Sequence: Synthetic oligonucleotide
  source 1..32: mol_type = other DNA
tcatacagatgatgaaggtaaagtcaaaatca

SEQ ID NO: 250 - DNA, 29 bp, synthetic construct
  misc_feature 1..29: note = Description of Artificial Sequence: Synthetic oligonucleotide
  source 1..29: mol_type = other DNA
tcatacagatgaaggtaaagtcaaaatca

SEQ ID NO: 251 - DNA, 42 bp, synthetic construct
  misc_feature 1..42: note = Description of Artificial Sequence: Synthetic oligonucleotide
  source 1..42: mol_type = other DNA
tcatacagatgatgtctacagatgaaggtaaagtcaaaatca

SEQ ID NO: 252 - DNA, 51 bp, synthetic construct
  misc_feature 1..51: note = Description of Artificial Sequence: Synthetic oligonucleotide
  source 1..51: mol_type = other DNA
tcatacagatgatgtctcatcatcaggagcgagaaggtaaagtcaaaatca

SEQ ID NO: 253 - DNA, 34 bp, synthetic construct
  misc_feature 1..34: note = Description of Artificial Sequence: Synthetic oligonucleotide
  source 1..34: mol_type = other DNA
gtcatcctcatcctgataaactgcaaaaggctga

SEQ ID NO: 254 - DNA, 606 bp, Homo sapiens
  source 1..606: mol_type = other DNA
gctggtgtctgggttctgtgccccttccccaccccagcccaccccaggtgtcctgtccattctcaggctggtcacatgggtggtcctagggtgtcccatgagagatgcaaagcgcctgaattttctgactcttcccatcagaccccccaaagacacatgtgacccaccaccccatctctgaccatgaggccaccctgaggtgctgggccctgggcttctaccctgcggagatcacactgacctggcagcgggatggcgaggaccaaactcaggacaccgagcttgtggagaccagaccagcaggagatagaaccttccagaagtgggcagctgtggtggtgccttctggagaagagcagagatacacatgccatgtacagcatgaggggctgccgaagcccctcaccctgagatggggtaaggagggggatgaggggtcatatctgttcatatctgttctcagggaaagcaggagcccttctggagcccttcagcagggtcagggcccctcatcttcccctcctttcccagagccatcttcccagtccaccatccccatcgtgggcattgttgctggcctggctgtcctagcagttgtggtcatcg

SEQ ID NO: 255 - DNA, 26 bp, Homo sapiens
  source 1..26: mol_type = other DNA
actaccacagctccttctctgagtgg

SEQ ID NO: 256 - DNA, 23 bp, synthetic construct
  misc_feature 1..23: note = Description of Artificial Sequence: Synthetic oligonucleotide
  source 1..23: mol_type = other DNA
actaccacagctcctctgagtgg

SEQ ID NO: 257 - DNA, 23 bp, Homo sapiens
  source 1..23: mol_type = other DNA
gtagttggagctggcggcgtagg

SEQ ID NO: 258 - DNA, 23 bp, synthetic construct
  misc_feature 1..23: note = Description of Artificial Sequence: Synthetic oligonucleotide
  source 1..23: mol_type = other DNA
gtagttggagctagcggcgtagg

SEQ ID NO: 259 - DNA, 23 bp, Homo sapiens
  source 1..23: mol_type = other DNA
gtagttggagctggtggcgtagg

SEQ ID NO: 260 - DNA, 23 bp, synthetic construct
  misc_feature 1..23: note = Description of Artificial Sequence: Synthetic oligonucleotide
  source 1..23: mol_type = other DNA
gtagttggagctagtggcgtagg

SEQ ID NO: 261 - DNA, 28 bp, synthetic construct
  misc_feature 1..28: note = Description of Artificial Sequence: Synthetic oligonucleotide
  source 1..28: mol_type = other DNA
ccatacattaaagatagtcatcttgggg

SEQ ID NO: 262 - DNA, 60 bp, Homo sapiens
  source 1..60: mol_type = other DNA
ccatacagtcagtatcaattctggaagaatttccagacattaaagatagtcatcttgggg

SEQ ID NO: 263 - DNA, 55 bp, Homo sapiens
  source 1..55: mol_type = other DNA
ccatacagtcagtatcaattctggaagaatttccagacattaaagatagtcatct

SEQ ID NO: 264 - DNA, 23 bp, synthetic construct
  misc_feature 1..23: note = Description of Artificial Sequence: Synthetic oligonucleotide
  source 1..23: mol_type = other DNA
ccatacattaaagatagtcatct

SEQ ID NO: 265 - DNA, 23 bp, Homo sapiens
  source 1..23: mol_type = other DNA
agatgactatctttaatgtctgg

SEQ ID NO: 266 - DNA, 23 bp, Homo sapiens
  source 1..23: mol_type = other DNA
agatgactatctttaatgtatgg

SEQ ID NO: 267 - DNA, 23 bp, synthetic construct
  misc_feature 1..23: note = Description of Artificial Sequence: Synthetic oligonucleotide
  source 1..23: mol_type = other DNA
gtagttggagctgatggcgtagg

SEQ ID NO: 268 - DNA, 23 bp, synthetic construct
  misc_feature 1..23: note = Description of Artificial Sequence: Synthetic oligonucleotide
  source 1..23: mol_type = other DNA
gtagttggagctggtagcgtagg

SEQ ID NO: 269 - DNA, 23 bp, synthetic construct
  misc_feature 1..23: note = Description of Artificial Sequence: Synthetic oligonucleotide
  source 1..23: mol_type = other DNA
gtagttggagctggtgacgtagg

SEQ ID NO: 270 - DNA, 23 bp, synthetic construct
  misc_feature 1..23: note = Description of Artificial Sequence: Synthetic oligonucleotide
  source 1..23: mol_type = other DNA
gtagttggagctaatggcgtagg

SEQ ID NO: 271 - DNA, 23 bp, synthetic construct
  misc_feature 1..23: note = Description of Artificial Sequence: Synthetic oligonucleotide
  source 1..23: mol_type = other DNA
gtagttggagctagtagcgtagg

SEQ ID NO: 272 - DNA, 23 bp, synthetic construct
  misc_feature 1..23: note = Description of Artificial Sequence: Synthetic oligonucleotide
  source 1..23: mol_type = other DNA
gtagttggagctagtgacgtagg

SEQ ID NO: 273 - DNA, 23 bp, Homo sapiens
  source 1..23: mol_type = other DNA
caaatgaatgatgcacatcatgg

SEQ ID NO: 274 - DNA, 23 bp, synthetic construct
  misc_feature 1..23: note = Description of Artificial Sequence: Synthetic oligonucleotide
  source 1..23: mol_type = other DNA
caaatgaatgatgcacgtcatgg

SEQ ID NO: 275 - DNA, 23 bp, synthetic construct
  misc_feature 1..23: note = Description of Artificial Sequence: Synthetic oligonucleotide
  source 1..23: mol_type = other DNA
caaatgaatgatgcatatcatgg

SEQ ID NO: 276 - DNA, 23 bp, synthetic construct
  misc_feature 1..23: note = Description of Artificial Sequence: Synthetic oligonucleotide
  source 1..23: mol_type = other DNA
caaatgaatgatgcgcatcatgg

SEQ ID NO: 277 - DNA, 23 bp, synthetic construct
  misc_feature 1..23: note = Description of Artificial Sequence: Synthetic oligonucleotide
  source 1..23: mol_type = other DNA
caaatgaatgatgtacatcatgg

SEQ ID NO: 278 - DNA, 23 bp, synthetic construct
  misc_feature 1..23: note = Description of Artificial Sequence: Synthetic oligonucleotide
  source 1..23: mol_type = other DNA
caaatgaatggtgcacatcatgg

SEQ ID NO: 279 - DNA, 23 bp, synthetic construct
  misc_feature 1..23: note = Description of Artificial Sequence: Synthetic oligonucleotide
  source 1..23: mol_type = other DNA
caaatgagtgatgcacatcatgg

SEQ ID NO: 280 - DNA, 23 bp, synthetic construct
  misc_feature 1..23: note = Description of Artificial Sequence: Synthetic oligonucleotide
  source 1..23: mol_type = other DNA
caaaagaatgatgcacatcatgg

SEQ ID NO: 281 - DNA, 23 bp, synthetic construct
  misc_feature 1..23: note = Description of Artificial Sequence: Synthetic oligonucleotide
  source 1..23: mol_type = other DNA
cgaatgaatgatgcacatcatgg

SEQ ID NO: 282 - DNA, 23 bp, synthetic construct
  misc_feature 1..23: note = Description of Artificial Sequence: Synthetic oligonucleotide
  source 1..23: mol_type = other DNA
caaatgaatgatgcatgtcatgg

SEQ ID NO: 283 - DNA, 23 bp, synthetic construct
  misc_feature 1..23: note = Description of Artificial Sequence: Synthetic oligonucleotide
  source 1..23: mol_type = other DNA
caaatgaatgatgcgcgtcatgg

SEQ ID NO: 284 - DNA, 23 bp, synthetic construct
  misc_feature 1..23: note = Description of Artificial Sequence: Synthetic oligonucleotide
  source 1..23: mol_type = other DNA
caaatgaatgatgtacgtcatgg

SEQ ID NO: 285 - DNA, 23 bp, synthetic construct
  misc_feature 1..23: note = Description of Artificial Sequence: Synthetic oligonucleotide
  source 1..23: mol_type = other DNA
caaatgaatggtgcacgtcatgg

SEQ ID NO: 286 - DNA, 23 bp, synthetic construct
  misc_feature 1..23: note = Description of Artificial Sequence: Synthetic oligonucleotide
  source 1..23: mol_type = other DNA
caaatgagtgatgcacgtcatgg

SEQ ID NO: 287 - DNA, 23 bp, synthetic construct
  misc_feature 1..23: note = Description of Artificial Sequence: Synthetic oligonucleotide
  source 1..23: mol_type = other DNA
caaaagaatgatgcacgtcatgg

SEQ ID NO: 288 - DNA, 23 bp, synthetic construct
  misc_feature 1..23: note = Description of Artificial Sequence: Synthetic oligonucleotide
  source 1..23: mol_type = other DNA
cgaatgaatgatgcacgtcatgg

SEQ ID NO: 289 - DNA, 23 bp, Homo sapiens
  source 1..23: mol_type = other DNA
atcataggtcgtcatgcttatgg

SEQ ID NO: 290 - DNA, 23 bp, synthetic construct
  misc_feature 1..23: note = Description of Artificial Sequence: Synthetic oligonucleotide
  source 1..23: mol_type = other DNA
atcataggttgtcatgcttatgg

SEQ ID NO: 291 - DNA, 23 bp, Homo sapiens
  source 1..23: mol_type = other DNA
atcataggtcgtcctgcttatgg

SEQ ID NO: 292 - DNA, 23 bp, synthetic construct
  misc_feature 1..23: note = Description of Artificial Sequence: Synthetic oligonucleotide
  source 1..23: mol_type = other DNA
atcataggttgtcctgcttatgg

SEQ ID NO: 293 - DNA, 23 bp, Homo sapiens
  source 1..23: mol_type = other DNA
ctggacaagaagagtacagtgcc

SEQ ID NO: 294 - DNA, 23 bp, synthetic construct
  misc_feature 1..23: note = Description of Artificial Sequence: Synthetic oligonucleotide
  source 1..23: mol_type = other DNA
ctggaaaagaagagtacagtgcc

SEQ ID NO: 295 - DNA, 23 bp, Homo sapiens
  source 1..23: mol_type = other DNA
actccatcgagatttcactgtag

SEQ ID NO: 296 - DNA, 23 bp, synthetic construct
  misc_feature 1..23: note = Description of Artificial Sequence: Synthetic oligonucleotide
  source 1..23: mol_type = other DNA
actccatcgagatttctctgtag

SEQ ID NO: 297 - RNA, 76 nt, synthetic construct
  source 1..76: mol_type = other RNA
gttttagagctagaaatagcaagttaaaataaggctagtccgttatcaacttgaaaaagtggcaccgagtcggtgc